European Patent Application EP 4 775 673 A1, published July 15, 2026. Title: 一种生物全合成紫杉醇前体物质巴卡亭III的方法、生物材料及应用. Applicant: 中国农业科学院深圳农业基因组研究所（岭南现代农业科学与技术广东省实验室深圳分中心）. The sequence listing filed with the application follows.

SEQUENCE LISTING (80 sequences)

SEQ ID NO: 1 - protein, 501 aa, unidentified
  source 1..501: note = T9H1 protein sequence; note (original language) = T9H1蛋白序列
MDSLSFLKSMEAKFGQVIHRDQSSSTALLSLAFTAALAIFLVLLFRFKSRPSTNFPPGNFGFPFIGETIQFLRALRSESPHMFFDERLKKFGRVFKTSLTGHPTAVFCGPAGNRFIYSNEHKLVQSSGPNSFVKLVGQQSIVTKTGEEHRIFRGVLNEFLGPHALQSYTPKMSSKIQENINKHWKGKDEVNMLPSIRQLVFSISSSLFFDINDEDQQEQLKTLLETILVGTLSVPLDIPGSNFRKALRARSKLDEILSRLIESRRKDMRSGIASTSKNLLSVLLAFKDERGNPLTDTEILDNFSFMLHASYDTTVSPTVCIFKLLSANPECYEKVVQEQLGILGNKKDGEEICWNDLKAMKYTWQAAQETMRLFPPAFGSFRKVIADIHHDGYIIPKGWKAMVTNYSTSRKEEYFDEPDKFKPSRFGDGKYVAPYTFLPFGAGIRICPGWEFAKLEMLLFIHHFVKNFSGYLPLDTKEKISGDPFPPLPKNGFPIKLFPRT

SEQ ID NO: 2 - protein, 489 aa, unidentified
  source 1..489: note = T9H2 protein sequence; note (original language) = T9H2蛋白序列
MDCFNFLTSMESSTALRLSLAFTAAVGIFLLLLFHYKRRPSINLPPGNFGFPFIGETIQFLRGLRSESPHVFFDERLKKFGSVFKTSLTGHPTAVFCGPAGNRLIFSNEDKLVQSSGPNSFVKLFGQQSIVSKTGEEHRIFRGALAQFLGPHALQSYTPKINSKIQENIDKKWKGKDEVKMLPLIRGLIFSIASSLFFDINDEDQQEQLHTLLETILLGTLSIPLDFPGSNFRKALKARSKLDEILSCLIKSRRKDMRSGIASTNQNLLSVLLTFKDERGNPLTDMEILDNFSVMLHASYDTTVSPTILLFKLLSANPECYEKVVQEQLGILGDKDGEEIVWNDLKCMKYTWQVVQETMRIFPPTFGSFRKVIADIHHDGYTIPKGWRVLVTNHSTSGKEEYFDEPDKFKPSRFEDGKYVAPYTFLPFGAGIRICPGWEFAKLEMLLFIHHFVKHFSGYIPIDTKEKVSGDPFPPLPNNGFPIKLLPRT

SEQ ID NO: 3 - protein, 499 aa, unidentified
  source 1..499: note = T9H3 protein sequence; note (original language) = T9H3蛋白序列
MDRFNLLRGIVSNLGEVIQLDSSPAIISLTLAAILGIIVLFIFRYNHRSSVKLPPGNLGFPFIGETVPFLRALRSETPQTFFDGRMKKFGPVFLTSLIGHPTVVFCGPAGNRLLLSNEDKLVNMTSPKSSRKVFGQNSIVTKRGEEHRIFRAALIRFLRPQAIQSYIGRMNSKVERHINEKWKGKDEVKALPLIRDLIFSIASSLFFDINDEHQQKRLHHLLETVLMGSMSVPLDFPGTPFRKAVQARSKLDEVLSCLIKSRRNDLRSGIASEDQDLLSVLLTFKDERGNPLADNEILDNFSVILHASYDTTVSPTVLLFKFLFSNPECYEKVVQEQLGIHGNKKEGEEINWNDLKAMKYTWQVVQETMRIFPPAFGAFRQAITDIHYDGYTVPKGYNILWTPYATHVKEEYFNEADKFMPSRFEEGKYVTPYTYLPFGAGLRVCPGWEFAKAEMLLIVHHFVRNFSSFFPVDPNEKISGDPFPPLPTNGFSMKLFPRS

SEQ ID NO: 4 - protein, 501 aa, unidentified
  source 1..501: note = T9H4 protein sequence; note (original language) = T9H4蛋白序列
MDSLSFLKSMEAKFGQVIHRDQSSSTALLSLAFTAALAIFLVLLFRFKSRPSTNFPPGNFGFPFIGETIQFLRALRSESPHMFFDERLKKFGRVFKTSLTGHPTAVFCGPAGNRFIYSNEHKLVQSSGPNSFVKLVGQQSIVTKTGEEHRIFRGVLNEFLGPHALQSYTPKMSSKIQENINKHWKGKDEVNMLPSIRQLVFSISSSLFFDINDEDQQEQLKTLLETILVGTLSVPLDIPGSNFRKALRARSKLDEILSRLIESRRKDMRSGIASTSKNLLSVLLAFKDERGNPLTDTEILDNFSFMLHASYDTTVSPTVCIFKLLSANPECYEKVVQEQLGILGNKKDGEEICWNDLKAMKYTWQAAQETMRLFPPAFGSFRKVIADILHDGYIIPKGWKAMVTNYSTSRKEEYFDEPDKFKPSRFGEGKYVAPYTFLPFGAGIRICPGWEFAKLEMLLFIHHFVKNFSGYLPLDTKEKISGDPFPPLPKNGFPIKLFPRT

SEQ ID NO: 5 - protein, 499 aa, unidentified
  source 1..499: note = T9H5 protein sequence; note (original language) = T9H5蛋白序列
MDRFNLLRGIVSNLGEVIQLDSSPAFISLTLAAILGIIVLFIFRYNHRSSVKLPPGNLGFPFIGETIPFLRALRSETPQTFFDGRMKKFGPVFLTSLIGHPTVVFCGPAGNRLLLSNEDKLVNMTSPKSSRKVFGQNSIVTKRGEEHRIFRAALTRFLRPQAIQSYIGRMNSKVERHINEKWKGKDEVKALPLIRDLIFSIASSLFFDINDEHQQKRLHHLLETVLMGSMSVPLDFPGTPFRKAVQARSKLDEILSCLIKSRRNDLRSGIASEDQDLLSVLLTFKDERGNPLADNEILDNFSVILHASYDTTVSPTVLLFKFLFSNSECYEKVVQEQLGIHGNKKEGEEINWNDLKAMKYTWQVVQETMRIFPPAFGAFRQAITDIHYDGYTVPKGYNILWTPYATHVKEEYFNEADKFMPSRFEEGKYVTPYTYLPFGAGLRVCPGWEFAKAEMLLIVHHFVRNFSSFFPVDPNEKISGDPFPPLPTNGFSMKLFPRS

SEQ ID NO: 6 - protein, 501 aa, unidentified
  source 1..501: note = T9H6 protein sequence; note (original language) = T9H6蛋白序列
MDSFSFLKSMEAKFGQVIHRDQSSSTALLSLAFTAAVAIFLVLLFRFKSRPSTNFPPGNFGFPFIGETIQFLRALRSESPHMFFDERLKKFGRVFKTSLTGHPTAVFCGPAGNRFIYSNEHKLVQSSGPNSFVKLVGQQSIVTKTGEEHRIFRGVLNEFLGPHALQSYTPKMSSKIQENINKHWKGKDEVNMLPSIRQLVFSISSSLFFDINDEDQQEQLKTLLETILVGTLSVPLDIPGSNFRKALRARSKLDEILSRLIESRRKDMRSGIASTSKNLLSVLLAFKDERGNPLTDTEILDNFSFMLHASYDTTVSPTVCIFKLLSANPECYEKVVQEQLGILGNKKDGEEICWNDLKAMKYTWQAAQETMRLFPPAFGSFRKVIADIHHDGYIIPKGWKAMVTNYSTSRKEEYFDEPDKFKPSRFGDGKYVAPYTFLPFGAGIRICPGWEFAKLEMLLFIHHFVKNFSGYLPLDTKEKISGDPFPPLPKNGFPIKLFPRT

SEQ ID NO: 7 - protein, 499 aa, unidentified
  source 1..499: note = T9H7 protein sequence; note (original language) = T9H7蛋白序列
MDRFNFVRDIVANLGEVIQLESSPAIISLTLAAILGIILLFIFRYNNRSSVKLPPGNLGFPFIGETIPFLRALRSETPQTFFDGRMKKFGPVFLTSLIGHPTVVFCGPAGNRLLLSNEDKLVNMTSPKSSRKVFGQNSIVTKRGEEHRIFRAALARFLRPQAIQSYIGRMNSKVERHINEKWKGKDEVKALPLIRYLIFSIASSLFFDINDEHQQKRLHHLLETVLMGSMSVPLDFPGTPFRKAVQARSKLDEILSCLIKSRRNDLRSGIASEDQDLLSVLLTFKDERGNPLADNEILDNFSVILHASYDTTVSPSVLLFKFLFSNPECYEKVVQEQLGIHGNKKEGEEINWNDLKAMKYTWQVVQETMRIFPPAFGAFRQAITDVHYDGYTVPKGYNILWTPYATHVKEEYFNEADKFMPSRFEEGKYVAPYTYLPFGAGLRVCPGWEFAKAEMLLIVHHFVRNFSSFFPVDPNEKISGDPFPPLPTNGFSMKLFPRS

SEQ ID NO: 8 - protein, 501 aa, unidentified
  source 1..501: note = T9H8 protein sequence; note (original language) = T9H8蛋白序列
MDSFSFLKSMEAKFGQVIHRDQSSSTVLLSLAFTAAVAIFLVLLFRFKSRPSTNFPPGNFGFPFIGETIQFLRALRSESPHRFFDERLKKFGNVFKTSLTGHPTAVFCGPAGNRFIYSNEHKLVQSSGPNSFVKLVGQQSIVTKTGEEHRIFRGVLNEFLGPHALQSYTPKMSSKIQENINKHWKGKDEVNMLPSIRQLVFSISSSLFFDINDEDQQEQLKTLLETILVGTLSVPLDIPGSNFRKALRARSKLDEILSRLIESRRKDMRSGIASTSKNLLSVLLAFKDERGNPLTDTEILDNFSFMLHASYDTTVSPTVCIFKLLSANPECYEKVVQEQLGILGNKKDGEEICWNDLKAMKYTWQAAQETMRLFPPAFGSFRKVIADIHHDGYIIPKGWKAMVTNYSTSRKEEYFDEPDKFKPSRFGDGKYVAPYTFLPFGAGIRICPGWEFAKLEMLLFIHHFVKNFSGYLPLDTKEKISGDPFPPLPKNGFPIKLFPRT

SEQ ID NO: 9 - protein, 499 aa, unidentified
  source 1..499: note = T9H9 protein sequence; note (original language) = T9H9蛋白序列
MDRFNLLRGIVSNLGEVIQLDSSPAIISLTLAAILGIIVLFIFRYNHRSSVKLPPGNLGFPFIGETIPFLQALRSETPQTFFDGRMKKFGPVFLTSLIGHPTVVFCGPAGNRLLLSNEDKLVNMTSPKSSRKVFGQNSIVTKRGEEHRIFRAALTRFLRPQAIQSYIGRMNSKVERHINEKWKGKDEVKALPLIRDLIFSIASSLFFDINDEHQQKRLHHLLETVLMGSMSVPLDFPGTPFRKAVQARSKLDEVLSCLIKSRRNDLRSGIASEDQDLLSVLLTFKDERGNPLADNEILDNFSVILHASYDTTVSPTVLLFKFLFSNPECYEKVVQEQLGIHGNKKEGEEINWNDLKAMKYTWQVVQETMRIFPPAFGAFRQAITDIHYDGYTVPKGYNILWTPYATHVKEEYFNEADKFMPSRFEEGKYVTPYTYLPFGAGLRVCPGWEFAKAEMLLIVHHFVRNFSSFFPVDPTEKISGDPFPPLPTNGFSMKLFPRS

SEQ ID NO: 10 - protein, 492 aa, unidentified
  source 1..492: note = T9H10 protein sequence; note (original language) = T9H10蛋白序列
MDSFNFPRGGVIQLGYSPAILSLTLAPILAILLLFFFRYTHRSSDKLPPGNLGFPFIGETIQLMRALRTETPQTFFDERVKKFGHVFKTSLIGYPTVVLSGPAGNRLLLSNEEKLVHSSSPKSTLKLFGQDSVLTKRGEEHRIFRAALARFLRPQALQGYVAKMNSEIQHHMNQKWKGKHQVKVLPLVRALIFNIASSFFFGITDEHLQERLHNLLEAILLGSMSVPLDFPGTRFRKALEARSKLDEILSSLIKKRRSDLLRSTSDNQDLLSVLLTFKDERGNPLTDKEILDNFSVMLHGSYETSVSPTVLVFKLLFSNPDCYEKVVQEQLGILCNKKEGEEISWNDLKTMKYTWQVVQETMRMFPPVFGSYRKAITDIHYDGYTIPKGWKIFWSPYTTHGKEEYFNEADKFMPSRFEEGKYVAPYTFLPFGAGVRVCPGWEFAKTEILLFVHHFVRTFSSYIPIDPKEKISGDPFPPLPTNGFSMKLFSRS

SEQ ID NO: 11 - protein, 492 aa, unidentified
  source 1..492: note = T9H11 protein sequence; note (original language) = T9H11蛋白序列
MDSFNFPRGGVIQLGYSPAILSLTLAPILAILLLFFFRYTHRSSDKLPPGNLGFPFIGETIQLMRALRTETPQTFFDERVKKFGHVFKTSLIGYPTVVLSGPAGNRLLLSNEEKLVHSSSPKSTLKLFGQDSVLTKRGEEHRIFRAALARFLRPQALQGYVAKMNSEIQHHMNQKWKGKHQVKVLPLVRALIFNIASSFFFGITDEHLQERLHNLLEAILLGSMSVPLDFPGTRFRKALEARSKLDEILSSLIKKRRSDLLRSTSDNQDLLSVLLTFKDERGNPLTDKEILDNFSVMLHGSYETSVSPTVLVFKLLFSNPDCYEKVVQEQLGILCNKKEGEEISWNDLKTMKYTWQVVQETMRMFPPVFGSYRKAITDIHYDGYTIPKGWNIFWSPYTTHGKEEYFNEADKFMPSRFEEGKYVAPYTFLPFGAGLRVCPGWEFAKTEILLFVHHFVTTFSSYIPIDPIEKISGDPFPPLPTDGFSMKLFTRS

SEQ ID NO: 12 - protein, 501 aa, unidentified
  source 1..501: note = T9H12 protein sequence; note (original language) = T9H12蛋白序列
MDSFSFLKSMEAKFGQVIHRDQSSSTALLSLAFTAAVAIFLVLLFRFKSRPSTNFPPGNFGFPFIGETIQFLRALRSESPHMFFDERLKKFGRVFKTSLTGHPTAVFCGPAGNRFIYSNEHKLVQSSGPNSFVKLVGQQSIVTKTGEEHRIFRGVLNEFLGPHALQSYTPKMSSKIQENINKHWKGKDEVNMLPSIRQLVFSISSSLFFDINDEDQQEQLKTLLETILVGTLSVPLDIPGSNFRKALRARSKLDEILSRLIESRRKDMRSGIASTSKNLLSVLLAFKDERGNPLTDTEILDNFSFMLHASYDTTVSPTVCIFKLLSANPECYEKVVQEQLGIHGNKKEGEEINWNDLKAMKYTWQAAQETMRLFPPAFGSFRKVIADIHHDGYIIPKGWKAMVTNYSTSRKEEYFDEPDKFKPSRFGDGKYVAPYTFLPFGAGIRICPGWEFAKLEMLLFIHHFVKNFSGYLPLDTKEKISGDPFPPLPKNGFPIKLFPRT

SEQ ID NO: 13 - protein, 491 aa, unidentified
  source 1..491: note = T9H13 protein sequence; note (original language) = T9H13蛋白序列
MNTFSFLPPNFLGFIQLQSILFLTLLALLLLCLFRYKTPSSAVKLPPGNLGFPFIGETIPFLRALHSETPQTFFDERMKRFGNVFVTSLIGQPIVVLCGPAGNRLLLSNEDKLVEMSPPKFSLKLIGQDSLLSKREDEHRTLRAALARFLRPQALQSYMGIMSSEIEQHINEKWKVKDEVKMLPLIRGLIFSIATTLFFDINDEHLKDRLHHLLETILVGTVSLPLDFPGTSFRKAVEARSKLDEILSSLIKSRRSDLHSGIVSDGQDLLTVLLTFKDERGNSLADNEILDNFSLMLHASYETSVSPTVLMFKLLSSNPECYDKLVQEQLGILANKKEGEDISWKDVKAMKYTWQVVQETMRIFPPAFGAFRQAITDIHYDGYTVPKGYNILWTPYATHVKEEYFNEADKFMPSRFEEGKYVAPYTYLPFGAGLRVCPGWEFAKAEMLLIVHHFVRNFSSFFPVDPNEKISGDPFPPLPTNGFSMKLFPRS

SEQ ID NO: 14 - protein, 491 aa, unidentified
  source 1..491: note = T9H14 protein sequence; note (original language) = T9H14蛋白序列
MNTFSFLPPNFLGFIQLQSILFLTLLALLLLCLFRYKTPSSAVKLPPGNLGFPFIGETIPFLRALHSETPQTFFDERMKRFGNVFVTSLIGQPIVVLCGPAGNRLLLSNEDKLVEMSPPKFSLKLIGQDSLLSKREDEHRTLRAALARFLRPQALQSYMGIMSSEIEQHINEKWKVKDEVKMLPLIRGLIFSIATTLFFDINDEHLKDRLHHLLETILVGTVSLPLDFPGTSFRKAVEARSKLDEILSSLIKSRRSDLHSGIVSDGQDLLTVLLTFKDERGNSLADNEILDNFSLMLHASYETSVSPTVLMFKLLSSNPECYDKLVQEQLGILANKKEGEDISWKDVKAMKYTWQVVQETMRIFPPGFGSYRKAITDIDYDGYTIPKGWTTLWTPYTTHGKEQYFHDPEQFRPSRFEEGERVAPYTFLPFGAGARICPGWEFAKTEILLFVHHFVKNFSSYHLVDPKEKVSGNPFPPLPNNGFSLKVFPRS

SEQ ID NO: 15 - DNA, 1506 bp, unidentified
  source 1..1506: mol_type = other DNA; note = T9H1 reading frame nucleotide sequence; note (original language) = T9H1读码框核苷酸序列
atggattccttaagttttctaaaaagcatggaagcgaaattcggccaagtcatacaccgggatcagtcttccagtactgctcttctgtccctcgcattcacagctgctcttgccatttttcttgtgttgctctttcgatttaaaagccggccctctactaatttccctccaggaaattttggcttccctttcattggagagacgatacagttcttgcgggcacttcgatcagaatcgcctcatatgttttttgatgagagattgaagaaatttgggcgtgtattcaagacgtcattaactgggcatcccacagctgtgttctgcgggcctgcgggaaaccggtttatttactcgaatgagcacaagctggtgcagtcgtctgggcccaactccttcgtcaaactggttgggcagcaatccatcgtgaccaaaacaggagaggagcaccgcatctttcgtggtgtcctgaacgagtttctggggcctcatgccttacagagttatacgcctaaaatgagttccaaaatccaggagaatatcaataagcattggaagggtaaagatgaagtgaacatgcttccttcgataagacagctcgtcttctccatttcaagcagcttgttttttgatattaatgatgaggatcaacaggaacaacttaaaactcttttagaaactattcttgttggaactttgtcggttcccctcgacattccaggatctaattttcgtaaagctcttcgggcgcgttccaagctggatgaaattctgtctcgtttaatcgaaagcagaagaaaagatatgcgttctgggatagcttctaccagtaaaaatctactgtcggtgctgctcgccttcaaagatgaaagagggaatccattgacggacacggagatcctcgacaacttttcttttatgcttcacgcctcatacgacaccaccgtttcgcccacggtttgtatatttaagctgctctccgccaatccagaatgctatgaaaaagtagttcaagaacaattgggaatacttggcaataaaaaggacggtgaagaaatctgttggaacgatctgaaagctatgaaatatacatggcaagcagctcaagaaacaatgaggcttttccctccagcgtttggatcatttcgcaaggtcatcgccgatattcatcatgatggctatataattcccaaaggatggaaagctatggtgacaaattacagtacaagtaggaaagaagagtacttcgatgaaccagacaaattcaagccttcaagatttggggatggaaagtatgtggctccgtacacgttcttacctttcggggcaggaatacgcatatgcccaggatgggagttcgctaagttggagatgttactgttcatccatcattttgtcaaaaatttcagcggatacctcccacttgacaccaaggaaaagatttccggagatccattccctcctctccccaaaaatggatttcccattaaactatttcccagaacctaa

SEQ ID NO: 16 - DNA, 1470 bp, unidentified
  source 1..1470: mol_type = other DNA; note = T9H2 reading frame nucleotide sequence; note (original language) = T9H2读码框核苷酸序列
atggattgcttcaattttctaacaagcatggagtcttccactgctcttcgactatccctcgccttcacagctgctgttggcattttccttctgttgctcttccattataaacgcaggccctctattaatcttcccccaggaaattttggcttccctttcattggagaaacgatacaattcttgcggggacttcgatcagaatcgcctcatgtgttttttgatgagagattgaagaaattcgggagtgtattcaagacgtcattaactggacatcccacagctgtgttctgcggtcctgcgggaaaccgcttaattttctcgaatgaggacaagctggtgcagtcgtcggggcccaactctttcgtcaaactgtttgggcagcaatccatcgtttccaaaacaggagaggagcatcgcatctttcgtggtgccctcgcccagtttctgggtcctcatgctttacagagttacacgcctaaaataaactccaaaatccaggagaatatcgataaaaaatggaagggcaaagatgaagtgaagatgcttcctttgataagagggctcatcttctccatcgcaagcagcttgtttttcgatattaatgatgaggatcaacaggaacaacttcatactcttttagaaactattcttctgggaacattgtcgattcctctcgactttccaggatctaattttcgtaaagctcttaaggcgcgttccaagctggatgaaattctttcttgtttgataaaaagcagaagaaaagatatgcgttctgggatagcttctaccaatcaaaatctgctgtcggtgctgctcaccttcaaagatgaaagagggaatccactgacggacatggagatcctcgacaacttttctgttatgcttcacgcctcatacgacaccactgtttcaccaacgatcttgttatttaagcttctctccgccaatccagaatgctatgaaaaagtagtccaagaacaactgggaatacttggcgataaggacggtgaagaaatcgtttggaacgatctgaaatgtatgaaatatacatggcaagtagttcaagaaacaatgaggatcttccctccaacgtttggatcatttcgcaaggttatcgccgatattcatcatgatggctacacaattccgaaaggatggagagttctggtgacaaatcacagtacaagtgggaaagaagagtacttcgatgaaccggacaaattcaagccttcaagatttgaggatggaaagtacgtagctccgtatacgttcttacctttcggggcaggcatacgcatatgcccaggatgggaattcgcaaagctggagatgttactgttcatccatcattttgttaaacatttcagtgggtacatcccaattgacaccaaggaaaaggtttccggagatccattccctcctctcccgaacaatggatttcccataaaactccttcccagaacctaa

SEQ ID NO: 17 - DNA, 1500 bp, unidentified
  source 1..1500: mol_type = other DNA; note = T9H3 reading frame nucleotide sequence; note (original language) = T9H3读码框核苷酸序列
atggatcgcttcaatttgctgagaggcatagtttcaaatttaggggaagtcattcaactggactcttcccctgctattatttcccttaccctcgcagctatccttggcattattgtcctctttatcttccgttataatcaccgatcttctgttaaacttccccctggaaatttaggcttccccttcattggggagaccgtaccattcttgcgggcgcttcgatcagaaacccctcaaacattttttgatgggagaatgaagaaattcggtcctgttttcctgacatcgctaattgggcatcccacagttgtattctgcgggcctgcgggaaatcgccttcttctctccaacgaggacaaactggtaaacatgacatcgcccaagtcttccagaaaagtgtttgggcagaattccattgtgaccaaaagaggcgaggagcatcgcatcttccgtgctgcacttatccgttttttgcgtccccaagccatacagagttatattggtagaatgaattccaaagtcgaacgtcatatcaacgaaaaatggaagggaaaagacgaagtgaaggcgcttcctttgataagagacctcatcttttccattgcaagcagtctgtttttcgatataaatgatgagcaccaacagaagcgacttcatcatctgttggaaaccgttcttatgggaagtatgtctgtcccgctcgactttccaggaactccttttcgtaaagctgttcaggcgcgatcaaagctggatgaagttctttcttgtttgataaaaagcagaagaaacgatctccgttcgggcatagcttctgaagatcaagatcttctctctgtgttgctcaccttcaaagatgaaagaggaaatccactcgccgacaacgagatcctggacaacttttctgttatacttcatgcctcgtatgacaccactgtttcacccactgttttgttatttaaattcctcttctccaatcctgaatgctatgaaaaagttgttcaagagcaattgggaatccatggcaataaaaaggagggggaagaaatcaattggaacgatctgaaagctatgaaatatacatggcaagtagttcaggaaacaatgaggattttccctccagcttttggagcttttcgccaagctatcaccgatattcactacgatggctatacagttccaaagggatacaatatattatggacaccttatgctacacatgtgaaagaagagtacttcaatgaagcggacaagttcatgccttcaagattcgaggaaggcaaatatgttaccccttacacatacttgccattcggagcaggcttgcgcgtatgtccaggatgggaatttgcaaaggcagagatgttactgatcgtccatcattttgttagaaacttcagcagctttttcccagtcgacccaaatgaaaaaatttcaggagatccattccctcctctccctaccaatggattttctatgaaactttttcccagatcctag

SEQ ID NO: 18 - DNA, 1506 bp, unidentified
  source 1..1506: mol_type = other DNA; note = T9H4 reading frame nucleotide sequence; note (original language) = T9H4读码框核苷酸序列
atggattccttaagttttctaaaaagcatggaagcgaaattcggccaagtcatacaccgggatcagtcttccagtactgctcttctgtccctcgcattcacagctgctcttgccatttttcttgtgttgctctttcgatttaaaagccggccctctactaatttccctccaggaaattttggcttccctttcattggagagacgatacagttcttgcgggcacttcgatcagaatcgcctcatatgttttttgatgagagattgaagaaatttgggcgtgtattcaagacgtcattaactgggcatcccacagctgtgttctgcgggcctgcgggaaaccggtttatttactcgaatgagcacaagctggtgcagtcgtctgggcccaactccttcgtcaaactggttgggcagcaatccatcgtgaccaaaacaggagaggagcaccgcatctttcgtggtgtcctgaacgagtttctggggcctcatgccttacagagttatacgcctaaaatgagttccaaaatccaggagaatatcaataagcattggaagggtaaagatgaagtgaacatgcttccttcgataagacagctcgtcttctccatttcaagcagcttgttttttgatattaatgatgaggatcaacaggaacaacttaaaactctgttagaaactattcttgttggaactttgtcggttcccctcgacattccaggatctaattttcgtaaagctcttcgggcgcgttccaagctggatgaaattctgtctcgtttaatcgaaagcagaagaaaagatatgcgttctgggatagcttctaccagtaaaaatctactgtcggtgctgctcgccttcaaagatgaaagagggaatccattgacggacacggagatcctcgacaacttttcttttatgcttcacgcctcatacgacaccaccgtttcgcccacggtttgtatatttaagctgctctccgccaatccagaatgctatgaaaaagtagttcaagaacaattgggaatacttggcaataaaaaggacggtgaagaaatctgttggaacgatctgaaagctatgaaatatacatggcaagcagctcaagaaacaatgaggcttttccctccagcgtttggatcatttcgcaaggtcatcgccgatattcttcatgatggctatataattcccaaaggatggaaagctatggtgacaaattacagtacaagtaggaaagaagagtacttcgatgaaccagacaaattcaagccttcaagatttggggaaggaaagtatgtggctccgtacacgttcttacctttcggggcaggaatacgcatatgcccaggatgggagttcgctaagttggagatgttactgttcatccatcattttgtcaaaaatttcagcggatacctcccacttgacaccaaggaaaagatttccggagatccattccctcctctccccaaaaatggatttcccattaaactatttcccagaacctaa

SEQ ID NO: 19 - DNA, 1500 bp, unidentified
  source 1..1500: mol_type = other DNA; note = T9H5 reading frame nucleotide sequence; note (original language) = T9H5读码框核苷酸序列
atggatcgcttcaatttgctgagaggcatagtttcaaatttaggggaagtcattcaactggattcttcccctgcttttatttcccttaccctcgcagctatccttggcattattgtcctctttatcttccgttataatcaccgatcttctgttaaacttccccctggaaatttaggcttccccttcattggggagaccataccattcttgcgggcccttcgatcagaaacccctcaaacattttttgatgggagaatgaagaaattcggtcctgttttcctgacatcgctaattgggcatcccacagttgtattctgcgggcctgcgggaaatcgccttcttctctccaacgaggacaaactggtaaacatgacatcgcccaagtcttccagaaaagtgtttgggcagaattccattgtgaccaaaagaggcgaggagcatcgcatcttccgtgctgcacttacccgttttttgcgtccccaagccatacagagttatattggtagaatgaattccaaagtcgaacgtcatatcaacgaaaaatggaagggaaaagacgaagtgaaggcgcttcctttgataagagacctcatcttttccattgcaagcagtctgtttttcgatataaatgatgagcaccaacagaagcgacttcatcatctgttggaaaccgttcttatgggaagtatgtctgttccgctcgactttccaggaactccttttcgtaaagctgttcaggcgcgatcaaagctggatgaaattctttcttgtttaataaaaagcagaagaaacgatctccgttcgggcatagcttctgaagatcaagatcttctctctgtgttgctcaccttcaaagatgaaagaggaaatccactcgccgacaacgagatcctggacaacttttctgttatacttcatgcctcgtatgacaccactgtttcacccactgttttgctatttaagttcctcttctccaattctgaatgctatgaaaaagtagttcaagagcaattgggaatccatggcaataaaaaggagggggaagaaatcaattggaacgatctgaaagctatgaaatatacatggcaagtagttcaggaaacaatgaggattttccctccagcttttggagcttttcgccaagctatcaccgacattcactacgatggctatacagttccaaagggatacaatatattatggacaccttatgctacacatgtgaaagaagagtacttcaatgaagcggacaagttcatgccttcaagattcgaggaaggcaaatatgttaccccttacacatacttgccattcggagcaggcttgcgcgtatgtccaggatgggaatttgcaaaggcagagatgttactgatcgtccatcattttgttagaaacttcagcagctttttcccagtcgacccaaatgaaaaaatttcaggagatccattccctcctctccctaccaatggattttctatgaaactttttcccagatcctag

SEQ ID NO: 20 - DNA, 1506 bp, unidentified
  source 1..1506: mol_type = other DNA; note = T9H6 reading frame nucleotide sequence; note (original language) = T9H6读码框核苷酸序列
atggattccttcagttttctaaaaagcatggaagcgaaattcggccaagtcatacaccgggatcagtcttccagtactgctcttctgtccctcgcattcacagctgctgttgccatttttcttgtgttgctctttcgatttaaaagccggccttctactaatttccctccaggaaattttggcttccctttcattggagagacgatacagttcttgcgggcacttcgatcagaatcgcctcatatgttttttgatgagagattgaagaagttcgggcgtgtattcaagacgtcattaactgggcaccccacagctgtgttctgcgggcctgcgggaaaccggtttatttactcgaatgagcacaagctggtgcagtcgtctgggcccaactcctttgtcaaactggttgggcagcaatccatcgtgaccaaaacaggagaggagcaccgcatctttcgtggtgtcctgaacgagtttctggggcctcatgccttacagagttatacgcctaaaatgagttccaaaatccaggagaatatcaataagcattggaagggtaaagatgaagtgaacatgcttccttcgataagacagctcgtcttctccatttcaagcagcttgttttttgatattaatgatgaggatcaacaggaacaacttaaaactcttttagaaactattcttgtgggaactttgtcggttcccctcgacattccaggatctaattttcgtaaagctcttcgggcgcgttccaagctggatgaaattctgtctcgtttaatcgaaagcagaagaaaagatatgcgttctgggatagcttctaccagtaaaaatctactgtcggtgctgctcgccttcaaagatgaaagagggaatccattgacggacacggagatcctcgacaacttttcttttatgcttcacgcctcatacgacaccaccgtttcgcccacagtttgtatatttaagctgctctccgccaatccagaatgctatgaaaaagtagttcaagaacaattgggaatacttggcaataaaaaggacggtgaagaaatctgttggaacgatctgaaagctatgaaatatacatggcaagcagctcaagaaacaatgaggcttttccctccagcgtttggatcatttcgcaaggtcatcgccgatattcatcatgatggctatataattcccaaaggatggaaagctatggtgacaaattacagtacaagtaggaaagaagagtacttcgatgaaccagacaaattcaagccttcaagatttggggatggaaagtatgtggctccgtacacgttcttacctttcggggcaggcatacgcatatgcccaggatgggagttcgctaagttggagatgttactgttcatccatcattttgtcaaaaatttcagcggatacctcccacttgacaccaaggaaaagatttccggagatccattccctcctctccccaaaaatggatttcccattaaactatttcccagaacctaa

SEQ ID NO: 21 - DNA, 1500 bp, unidentified
  source 1..1500: mol_type = other DNA; note = T9H7 reading frame nucleotide sequence; note (original language) = T9H7读码框核苷酸序列
atggatcgcttcaattttgtgagagacatagttgcaaatttaggggaagtaattcaactggagtcttcccctgctattatttcccttaccctcgcagctatccttggcattattcttctttttatcttccgttataataaccgatcctctgttaaacttccccctggaaatttaggcttccccttcattggggagaccataccattcttgcgggcgcttcgatcagaaacccctcaaacattttttgatgggagaatgaagaaattcggccctgttttcctgacttcgctaattgggcatcccacagttgtattctgcgggcctgcgggaaatcgccttcttctctccaacgaggacaaactagtaaacatgacatcgcccaagtcttccagaaaagtgtttgggcagaattccattgtgaccaaaagaggcgaggagcatcgcatcttccgtgctgcacttgcccgttttttgcgtccccaagccatacagagttatattggtagaatgaattccaaagtcgaacgtcatatcaacgaaaaatggaagggaaaagacgaagtgaaggcgcttcctttgataagatacctcatcttttccattgcaagcagtctgtttttcgatataaatgatgagcaccaacagaagcgacttcatcatctgttggaaaccgttcttatgggaagtatgtctgttccgctcgactttccaggaactccttttcgtaaagctgttcaggcgcgatcaaagctggatgaaattctttcttgtttgataaaaagcagaagaaacgatctccgttcgggcatagcttctgaagatcaagatcttctctctgtgttgctcaccttcaaagatgaaagaggaaatccactcgccgacaacgagatcctggacaacttttctgttatacttcatgcctcgtatgacaccactgtttcacccagtgttttgctatttaagttcctcttctccaatcctgaatgctatgaaaaagtagttcaagagcaattgggaatccatggcaataaaaaggagggggaagaaatcaattggaacgatctgaaagctatgaaatatacatggcaagtagttcaggaaacaatgaggattttccctccagcttttggagcttttcgccaagctatcaccgacgttcactacgatggctatacagttccaaagggatacaatatattatggacaccttatgctacacatgtgaaagaagagtacttcaatgaagcggacaagttcatgccttcaagattcgaggaaggcaaatatgttgccccttacacatacttgccattcggagcaggcttgcgcgtatgtccaggatgggaatttgcaaaggcagagatgttactgatcgtccatcattttgttagaaacttcagcagctttttcccagtcgacccaaatgaaaaaatttcaggagatccattccctcctctccctaccaatggattttctatgaaactttttcccagatcctag

SEQ ID NO: 22 - DNA, 1506 bp, unidentified
  source 1..1506: mol_type = other DNA; note = T9H8 reading frame nucleotide sequence; note (original language) = T9H8读码框核苷酸序列
atggattccttcagttttctaaaaagcatggaagcgaaatttggccaagtcatccaccgggatcagtcttccagtactgttcttctgtccctcgcattcacagctgctgttgccatttttcttgtgttgctctttcgatttaaaagccggccctctactaatttccctccaggaaattttggcttccctttcattggagagacgatacagttcttgcgggcacttcgatcagaatcgcctcataggttttttgatgagagattgaagaaatttgggaatgtattcaagacgtcattaactgggcatcccacagctgtgttctgcgggcctgcgggaaaccggtttatttactcgaatgagcacaagctggtgcagtcgtctgggcccaactccttcgtcaaactggttgggcagcaatccatcgtgaccaaaacaggagaggagcatcgcatctttcgtggtgtcctgaacgagtttctggggcctcatgccttacagagttatacgcctaaaatgagttccaaaatccaggagaatatcaataagcattggaagggtaaagatgaagtgaacatgcttccttcgataagacagctcgtcttctccatttcaagcagcttgttttttgatattaatgatgaggatcaacaggaacaacttaaaactcttttagaaactattcttgttggaactttgtcggttcccctcgacattccaggatctaattttcgtaaagctcttcgggcgcgttccaagctggatgaaattctgtctcgtttaatcgaaagcagaagaaaagatatgcgttctgggatagcttctaccagtaaaaatctactgtcggtgctgctcgccttcaaagatgaaagagggaatccattgacggacacggagatcctcgacaacttttcttttatgcttcacgcctcatacgacaccaccgtttcgcccacggtttgtatatttaagctgctctccgccaatccagaatgctatgaaaaagtagttcaagaacaattgggaatacttggcaataaaaaggacggtgaagaaatctgttggaacgatctgaaagctatgaaatatacatggcaagcagctcaagaaacaatgaggcttttccctccagcgtttggatcatttcgcaaggtcatcgccgatattcatcatgatggctatataattcccaaaggatggaaagctatggtgacaaattacagtacaagtaggaaagaagagtacttcgatgaaccagacaaattcaagccttcaagatttggggatggaaagtatgtggctccgtacacgttcttacctttcggggcaggcatacgcatatgcccaggatgggagttcgctaagttggagatgttactgttcatccatcattttgtcaaaaatttcagcggatacctcccacttgacaccaaggaaaagatttccggagatccattccctcctctccccaaaaatggatttcccattaaactatttcccagaacctaa

SEQ ID NO: 23 - DNA, 1500 bp, unidentified
  source 1..1500: mol_type = other DNA; note = T9H9 reading frame nucleotide sequence; note (original language) = T9H9读码框核苷酸序列
atggatcgcttcaatttgctgagaggcatagtttcaaatttaggggaagtcattcaactggactcttcccctgctattatttcccttaccctcgcagctatccttggcattattgtcctctttatcttccgttataatcaccgatcttctgttaaacttccccctggaaatttaggcttccccttcattggggagaccataccattcttgcaggcgcttcgatcagaaacccctcaaacattttttgatgggagaatgaagaaattcggtcctgttttcctgacatcgctaattgggcatcccacagttgtattctgcgggcctgcgggaaatcgccttcttctctccaacgaggacaaactggtaaacatgacatcgcccaagtcttccagaaaagtgtttgggcagaattccattgtgaccaaaagaggcgaggagcatcgcatcttccgtgctgcacttacccgttttttgcgtccccaagccatacagagttatattggtagaatgaattccaaagtcgaacgtcatatcaacgaaaaatggaagggaaaagacgaagtgaaggcgcttcctttgataagagacctcatcttttccattgcaagcagtctgtttttcgatataaatgatgagcaccaacagaagcgacttcatcatctgttggaaaccgttcttatgggaagtatgtctgttccgctcgactttccaggaactccttttcgtaaagctgttcaggcgcgatcaaagctggatgaagttctttcttgtttgataaaaagcagaagaaacgatctccgttcgggcatagcttctgaagatcaagatcttctctctgtgttgctcaccttcaaagatgaaagaggaaatccactcgccgacaacgagatcctggacaacttttctgttatacttcatgcctcgtatgacaccactgtttcacccactgttttgctatttaagttcctcttctccaatcctgaatgctatgaaaaagtagttcaagagcaattgggaatccatggcaataaaaaggagggggaagaaatcaattggaacgatctgaaagctatgaaatatacatggcaagtagttcaggaaacaatgaggattttccctccagcttttggagcttttcgccaagctatcaccgatattcactacgatggctatacagttccaaagggatacaatatattatggacaccttatgctacacatgtgaaagaagagtacttcaatgaagcggacaagttcatgccttcaagattcgaggaaggcaaatatgttaccccttacacatacttgccattcggagcaggcttgcgcgtatgtccaggatgggaatttgcaaaggcagagatgttactgatcgtccatcattttgttagaaacttcagcagctttttcccagtcgacccaactgaaaaaatttcaggagatccattccctcctctccctaccaatggattttctatgaaactttttcccagatcctag

SEQ ID NO: 24 - DNA, 1479 bp, unidentified
  source 1..1479: mol_type = other DNA; note = T9H10 reading frame nucleotide sequence; note (original language) = T9H10读码框核苷酸序列
atggatagcttcaatttcccgagagggggagtcattcagctgggttattcccctgctattctttcccttaccctcgcacctattcttgccattctcctcctcttcttcttccgttacactcaccgatcctctgataaacttcccccgggaaatttagggtttcctttcattggggagactatacagttaatgcgggcacttcgaacagaaacacctcagacgtttttcgatgagagagtgaagaagttcggtcatgttttcaagacttcgctcattgggtatcccacagttgtactgagtggacctgcgggaaacaggttacttctgtcgaacgaggagaagctggtgcattcgtcatcgcccaagtctaccctgaaattgttcgggcaggattctgttctgaccaaaagaggcgaggagcatcgtatcttccgtgccgcacttgcccgcttcttgcgaccccaagctttacagggttatgttgccaaaatgaattcagaaattcaacatcatatgaatcaaaaatggaagggaaaacatcaagtgaaggtgcttcctttggtaagagcgcttatcttcaacattgcaagcagcttttttttcggtataactgacgaacacctacaggaacgacttcataaccttttggaagctattcttctgggaagtatgtctgttccgctcgactttccaggcactcgttttcgtaaagctcttgaggcgcggtcgaagctggacgaaattctttcttctttgataaaaaagagaagaagcgatcttctgcgttcaacttctgacaatcaagatcttctttctgtgttgctcaccttcaaagatgaaagagggaatccactgacggacaaggagatccttgacaatttttctgtcatgcttcatggctcgtatgagaccagtgtttcacccacggttttggtgtttaagcttctcttctcaaatcctgattgctatgagaaagtagttcaagagcaattgggaatcctgtgcaataaaaaggagggagaagaaatcagctggaacgatctgaaaactatgaaatatacatggcaagttgtgcaggaaactatgaggatgttccctccagtttttggatcgtatcgcaaggctatcaccgatatccattatgatgggtatacaattccaaaaggatggaaaatattctggtcaccttatactacacacgggaaagaagagtacttcaatgaagcggacaagttcatgccttcaagattcgaggaaggcaaatatgttgctccttacacattcttgccattcggagcaggtgtccgcgtatgtccagggtgggaatttgcaaagaccgagatattactgttcgtccatcattttgttagaactttcagcagctacatcccaattgaccccaaagagaaaatttcaggggatccatttcctcctctgcctaccaatggattttccatgaaacttttttccagatcttaa

SEQ ID NO: 25 - DNA, 1479 bp, unidentified
  source 1..1479: mol_type = other DNA; note = T9H11 reading frame nucleotide sequence; note (original language) = T9H11读码框核苷酸序列
atggatagcttcaatttcccgagagggggagtcattcagctgggttattcccctgctattctttcccttaccctcgcacctattcttgccattctcctcctcttcttcttccgttacactcaccgatcctctgataaacttcccccgggaaatttagggtttcctttcattggggagactatacagttaatgcgggcacttcgaacagaaacacctcagacgtttttcgatgagagagtgaagaagttcggtcatgttttcaagacttcgctcattgggtatcccacagttgtactgagtggacctgcgggaaacaggttacttctgtcgaacgaggagaagctggtgcattcgtcatcgcccaagtctaccctgaaattgttcgggcaggattctgttctgaccaaaagaggcgaggagcatcgtatcttccgtgccgcacttgcccgcttcttgcgaccccaagctttacagggttatgttgccaaaatgaattcagaaattcaacatcatatgaatcaaaaatggaagggaaaacatcaagtgaaggtgcttcctttggtaagagcgcttatcttcaacattgcaagcagcttttttttcggtataactgacgaacacctacaggaacgacttcataaccttttggaagctattcttctgggaagtatgtctgttccgctcgactttccaggcactcgttttcgtaaagctcttgaggcgcggtcgaagctggacgaaattctttcttctttgataaaaaagagaagaagcgatcttctgcgttcaacttctgacaatcaagatcttctttctgtgttgctcaccttcaaagatgaaagagggaatccactgacggacaaggagatccttgacaatttttctgtcatgcttcatggctcgtatgagaccagtgtttcacccacggttttggtgtttaagcttctcttctcaaatcctgattgctatgagaaagtagttcaagagcaattgggaatcctgtgcaataaaaaggagggagaagaaatcagctggaacgatctgaaaactatgaaatatacatggcaagttgtgcaggaaactatgaggatgttccctccagtttttggatcgtatcgcaaggctatcaccgatatccattatgatgggtatacaattccaaaaggatggaatatattctggtcaccttatactacacacgggaaagaagaatacttcaatgaagcggacaagttcatgccttcgagattcgaggaaggcaaatatgttgctccttacacattcttgccattcggagcaggtctgcgcgtatgtccaggatgggaatttgcaaagaccgagatattactgttcgtccatcattttgttacaactttcagcagctacatcccaattgaccccatagagaaaatttcaggggatccattccctcctctgcccaccgatggattttccatgaaactttttaccagatcttaa

SEQ ID NO: 26 - DNA, 1506 bp, unidentified
  source 1..1506: mol_type = other DNA; note = T9H12 reading frame nucleotide sequence; note (original language) = T9H12读码框核苷酸序列
atggattccttcagttttctaaaaagcatggaagcgaaattcggccaagtcatacaccgggatcagtcttccagtactgctcttctgtccctcgcattcacagctgctgttgccatttttcttgtgttgctctttcgatttaaaagccggccttctactaatttccctccaggaaattttggcttccctttcattggagagacgatacagttcttgcgggcacttcgatcagaatcgcctcatatgttttttgatgagagattgaagaaatttgggcgtgtattcaagacgtcattaactgggcatcccacagctgtgttctgcgggcctgcgggaaaccggtttatttactcgaatgagcacaagctggtgcagtcgtctgggcccaactcctttgtcaaactggttgggcagcaatccatcgtgaccaaaacaggagaggagcaccgcatctttcgtggtgtcctgaacgagtttctggggcctcatgccttacagagttatacgcctaaaatgagttccaaaatccaggagaatatcaataagcattggaagggtaaagatgaagtgaacatgcttccttcgataagacagctcgtcttctccatttcaagcagcttgttttttgatattaatgatgaggatcaacaggaacaacttaaaactcttttagaaactattcttgtgggaactttgtcggttcccctcgacattccaggatctaattttcgtaaagctcttcgggcgcgttccaagctggatgaaattctgtctcgtttaatcgaaagcagaagaaaagatatgcgttctgggatagcttctaccagtaaaaatctactgtcggtgctgctcgccttcaaagatgaaagagggaatccattgacggacacggagatcctcgacaacttttcttttatgcttcacgcctcatacgacaccaccgtttcgcccacagtttgtatatttaagctgctctccgccaatccagaatgctatgaaaaagtagttcaagagcaattgggaatacatggcaataaaaaggagggggaagaaatcaattggaacgatctgaaagctatgaaatatacatggcaagcagctcaagaaacaatgaggcttttccctccagcgtttggatcatttcgcaaggtcatcgccgatattcatcatgatggctatataattcccaaaggatggaaagctatggtgacaaattacagtacaagtaggaaagaagagtacttcgatgaaccagacaaattcaagccttcaagatttggggatggaaagtatgtggctccgtacacgttcttacctttcggggcaggcatacgcatatgcccaggatgggagttcgctaagttggagatgttactgttcatccatcattttgtcaaaaatttcagcggatacctcccacttgacaccaaggaaaagatttccggagatccattccctcctctccccaaaaatggatttcccattaaactatttcccagaacctaa

SEQ ID NO: 27 - DNA, 1476 bp, unidentified
  source 1..1476: mol_type = other DNA; note = T9H13 reading frame nucleotide sequence; note (original language) = T9H13读码框核苷酸序列
atgaataccttcagtttcctgcctccaaatttcctcgggttcattcaactccagtctattctattccttacccttcttgcccttcttcttctctgcctcttccgatataaaaccccgtcctctgctgttaaacttccccctggaaacttagggttccctttcattggggagaccataccattcttgagggcacttcactcagaaacaccgcaaacctttttcgatgagagaatgaagagattcggtaatgttttcgtgacttcgctaattggacagccaatagttgtactctgcgggcctgccggaaaccgcttactactctccaacgaagacaagctggtggaaatgtcaccacccaagttttcgctgaagctgatcggccaggattcccttctgtccaaaagagaagacgagcatcgcaccctacgcgctgcactcgctcgctttctgcgaccccaagcccttcagagttatatgggtataatgagttcagaaatcgaacagcatatcaatgaaaaatggaaggtaaaagatgaagtgaagatgcttcctttgataagaggacttatcttctccattgcaaccaccttgtttttcgatatcaatgatgagcacctcaaggatcgccttcatcaccttttggaaactattcttgtgggaactgtgtctcttccgctcgacttcccaggaacttcttttcgtaaagctgttgaggcgcggtcgaagctcgatgaaattctttcttctttaataaaaagcagaagaagcgatctgcattcaggcatagtttctgatggtcaagatctgctcacagtcttgctcaccttcaaagacgaaagagggaattcactcgccgataacgagatcctcgacaacttttctcttatgcttcacgcctcctatgagaccagtgtttcaccaacggttttgatgtttaagctgctgtcctccaatcctgaatgttatgacaaactagttcaagagcaattgggaatacttgccaataaaaaggagggagaagacatcagctggaaggatgtgaaagctatgaaatatacatggcaagtagttcaggaaacaatgaggattttccctccagcttttggagcttttcgccaagctatcaccgacattcactacgatggctatacagttccaaagggatacaatatattatggacaccttatgctacacatgtgaaagaagagtacttcaatgaagcggacaagttcatgccttcaagattcgaggaaggcaaatatgttgccccttacacatacttgccattcggagccggcttgcgcgtatgtccaggatgggaatttgcaaaggcagagatgttactgatcgtccatcattttgttagaaacttcagcagctttttcccagtcgacccaaatgaaaaaatttcaggagatccattccctcctctccctaccaatggattttccatgaaactttttcccagatcttaa

SEQ ID NO: 28 - DNA, 1476 bp, unidentified
  source 1..1476: mol_type = other DNA; note = T9H14 reading frame nucleotide sequence; note (original language) = T9H14读码框核苷酸序列
atgaataccttcagtttcctgcctccaaatttcctcgggttcattcaactccagtctattctattccttacccttcttgcccttcttcttctctgcctcttccgatataaaaccccgtcctctgctgttaaacttccccctggaaacttagggttccctttcattggggagaccataccattcttgagggcacttcactcagaaacaccgcaaacctttttcgatgagagaatgaagagattcggtaatgttttcgtgacttcgctaattggacagccaatagttgtactctgcgggcctgccggaaaccgcttactactctccaacgaagacaagctggtggaaatgtcaccacccaagttttcgctgaagctgatcggccaggattcccttctgtccaaaagagaagacgagcatcgcaccctacgcgctgcactcgctcgctttctgcgaccccaagcccttcagagttatatgggtataatgagttcagaaatcgaacagcatatcaatgaaaaatggaaggtaaaagatgaagtgaagatgcttcctttgataagaggacttatcttctccattgcaaccaccttgtttttcgatatcaatgatgagcacctcaaggatcgccttcatcaccttttggaaactattcttgtgggaactgtgtctcttccgctcgacttcccaggaacttcttttcgtaaagctgttgaggcgcggtcgaagctcgatgaaattctttcttctttaataaaaagcagaagaagcgatctgcattcaggcatagtttctgatggtcaagatctgctcacagtcttgctcaccttcaaagacgaaagagggaattcactcgccgataacgagatcctcgacaacttttctcttatgcttcacgcctcctatgagaccagtgtttcaccaacggttttgatgtttaagctgctgtcctccaatcctgaatgttatgacaaactagttcaagagcaattgggaatacttgccaataaaaaggagggagaagacatcagctggaaggatgtgaaagctatgaaatatacatggcaagtagttcaggaaacaatgaggatattccctccaggttttggatcatatcgtaaggcgatcaccgatattgattatgatggttatacaattccaaaaggatggacaactttatggactccttatactacacatgggaaagaacagtacttccatgatcccgaacaattcaggccttcaagatttgaagaaggagaacgtgtagctccttacacattcttaccattcggagcaggcgcgcgcatatgtccaggatgggaattcgcaaagacagagatattactgttcgtccatcattttgttaaaaatttcagtagctaccacttagttgaccccaaggaaaaagtatcagggaatccattccctcctctccctaacaatggattttctctgaaagtatttcccagatcgtaa

SEQ ID NO: 29 - protein, 507 aa, unidentified
  source 1..507: note = TOT1 protein sequence; note (original language) = TOT1蛋白序列
MVHVLQVVKMDRVREIFNGSSGSPAGIPHSVITAGVGAIIIILLSLLLLRRSSKRGDSSHPPGNSGLPFIGETLSFTKAFKSNTLAEFFEERVKKFGNVFKISIIGPPTVVMCGNEGNRFIFANEEKLVHLSWSGRYAKILGGDSVSMKRGDDHRSVRAAFAGFLSPASLPIYISKMSAQIQDHINQKWKGKDVIAVVPLVKELVFNVSYNLFFSINDSEELHRLHKIFETIVEGHVSMPIDLPGFTFHRALQGRAKLKKVFSSLIERRRSDLSSGLASANQDLISVLLTYKDDRGYTMTHDELLDNFLSLLESSYDSVNSPMACIFKLLYANPECYEKVVQEQLGILSGKKEGQEISWKDLRSMKYTWQVLQETLRLYTQVAGIFRKAMTVIHYDGHTIPKGWQLLWATQTTHLNDKYFSEPEKFMPSRFDEEGNNVIPYSFVPFGGGRRMCPGWEFGKMEILLFVHHFVKAFSGFTPIDPDEKITGNPFPHLPANGFSIKPTPRS

SEQ ID NO: 30 - protein, 507 aa, unidentified
  source 1..507: note = TOT2 protein sequence; note (original language) = TOT2蛋白序列
MVHVLQVVKMDRVSEIFNGSSGSPAGIPHSVITAGVGAIIIILLSLVLLRRSSKRGDSSHPPGNSGLPFIGETLSFTKAFKSNTLAEFFEERVKKFGNVFKISIIGPPTVVMCGNEGNRFIFANEEKLMHLSWSGRYAKILGGESVSMKRGDDHRSVRAAFAGFLSPSALPLYVAKMSAQIQNHINEKWKGRDVIAVVPLVKELVFNVSSNLFFSMNDSEELHRLHQIFETIVDGHVSMPIDLPGFTFHKALQGRAKLKKVYSSLIERRRSDLSSGLASANQDLISVLLTYKDDRGYTMTHDELLDNFLSLIESSYDSINSPMACIFKLLYANPECYEKVVQEQLGILSGKKEGEEISWKDLRSMKYTWQAIQETLRIYTQVAGIFRKAMTDIHYDGHTIPKGWQLLWATQTTHLNDKYFSEPEKFMPSRFDEEGNNVIPYSFVPFGGGRRMCPGWEFGKMEILLFVHHFVKTFSGFTPIDPNEKITGNPFPHLPANGFLIKPILRS

SEQ ID NO: 31 - protein, 507 aa, unidentified
  source 1..507: note = TOT3 protein sequence; note (original language) = TOT3蛋白序列
MVHVLHVVKMDRVREIFNGSSGSPAGIPHSVITAGVGAIIIILLSLLLLRRSSKRGDSSHPPGNSGLPFIGETLSFTKAFKSNTLAEFFEERVKKFGNVFKISIIGPPTVVMCGNEGNRFIFANEEKLMHLSWSGRYAKILGGESVSMKRGDDHRSVRAAFAGFLSSASLPVYISKMSAQIQDHINEKWKGKDVIAVVPLVKELVFNVSYNLFFSINDSEELHRLHKIFETIVEGHLSMPIDLPGFTFHRALQGRAKLKKVFSSLIERRRSDLSSGLASANQDLISVLLTYKDDRGYTMTHDELLDNFLSLLEGSYDSINSPMACIFKLLYDNPECYEKVVQEQLGILSGKKEGQEISWKDLRSMKYTWQVLQETLRLYTQVAGIFRKAMTDIHYDGHTIPKGWQLLWANQTTHLNDKYFSEPEKFMPSRFDEEGNNMIPYSFVPFGGGRRMCPGWEFGKMEILLFVHHFVKTFSGFTPIDPNEKITGNPFPHLPANGFLIKPILRS

SEQ ID NO: 32 - protein, 507 aa, unidentified
  source 1..507: note = TOT4 protein sequence; note (original language) = TOT4蛋白序列
MVHVLQVVKMDRVSEIFNGSSGSPAGIPHSVITAGVGAIIIILLSLVLLRRSSKRGDSSHPPGNSGLPFIGETLSFTKAFKSNTLAEFFEERVKKFGNVFKISIIGPPTVVMCGNEGNRFIFANEEKLMHLSWSGRYAKILGGESVSMKRGDDHRSVRAAFAGFLSPSALPLYVAKMSAQIQNHINEKWKGRDVIAVVPLVKELVFNVSSNLFFSMNDSEELHRLHQIFETIVDGHVSMPIDLPGFTFHKALQGRAKLKKVYSSLIERRRSDLSSGLASANQDLISVLLTYKDDRGYTMTHDELLDNFLSLIESSYDSVNSPMACIFKLLYANPECYEKVVQEQLGILSGKKEGQEISWKDLRSMKYTWQVLQETLRLYTQVAGIFRKAMTVIHYDGHTIPKGWQLLWATQTTHLNDKYFSEPQKFMPSRFDEEGNNVIPYSFVPFGGGRRMCPGWEFGKMEILLFVHHFVKAFSGFTPIDPDEKITGNPFPHLPANGFLIKPILRS

SEQ ID NO: 33 - protein, 493 aa, unidentified
  source 1..493: note = TOT5 protein sequence; note (original language) = TOT5蛋白序列
MDTVRELNGGSGSSGIPLSLITAAVGAIIILSLLLLRRSKRGNSSHPPGNSGLPFIGETLSFTKAFKSNTLDQFFEERVKKFGQVFKLSVIGPPTVAMCGPEGNRFVFANEEKLVHLSWSGRYAKILGGDSVSMKRGDDHRSVRAAFAGFLSPASLPVYISKMSAQIQDHINEKWKGKDVIAVVPLVKELVFNVSYNLFFSINDSEELHRLHKIFETIVEGHVSMPIDLPGFTFHRALQGRAKLKKVFSSLIERRRSDLSSGLASANQDLISVLLTYKDDRGYTMTHDELLDNFLSLLEASYDSVNSPMACIFKLLYANPECYEKVVQEQLGILSGKKEGQEISWKDLRSMKYTWQVLQETLRLYTQVAGIFRKAMTDIHYNGHTIPKGWQLLWATQTTHLNDKYFSEPEKFMPSRFDEEGNNVIPYSFVPFGGGRRMCPGWEFGKMEILLFVHHFVKAFSGFTPIDPDEKITGNPFPHLPANGFSIKPTPRS

SEQ ID NO: 34 - protein, 507 aa, unidentified
  source 1..507: note = TOT6 protein sequence; note (original language) = TOT6蛋白序列
MVHVLQVVKMDRVSEIFNGSSGSPAGIPHSVITAGVGAIIIILLSLVLLRRSSKRGDSSHPPGNSGLPFIGETLSFTKAFKSNTLAEFFEERVKKFGNVFKISIIGPPTVVMCGNEGNRFIFANEEKLMHLSWSGRYAKILGGESVSMKRGDDHRSVRAAFAGFLSPSALPLYVAKMSAQIQNHINEKWKGRDVIAVVPLVKELVFNVSSNLFFGMNDSEELHRLHQIFETIVDGHVSMPIDLPGFTFHKALQGRAKLKKVYSSLIERRRSDLSSGLASANQDLISVLLTYKDDRGYTMTHVELLDNFLSLIESSYDSINSPMACIFKLLYANPECYEKVVQEQLGILSGKKEGEEISWKDLRSMKYTWQAIQETLRIYTQVAGIFRKAMTDIHYDGHTIPKGWQLLWATQTTHLNDKYFSEPEKFMPSRFDEEGNNVIPYSFVPFGGGRRMCPGWEFGKMEILLFVHHFVKTFSGFTPIDPNEKITGNPFPHLPANGFLIKPILRS

SEQ ID NO: 35 - protein, 507 aa, unidentified
  source 1..507: note = TOT7 protein sequence; note (original language) = TOT7蛋白序列
MVHVLQVVKMYRVSEIFNGSSGSPAGIPHSVITAGVGAIIIILLSLVLLRRSSKRGDSSHPPGNSGLPFIGETLSFTKAFKSNTLAEFFEERVKKFGNVFKISIIGPPTVVMCGNEGNRFIFANEEKLMHLSWSGRYAKILGGESVSMKRGDDHRSVRAAFAGFLSPSALPLYVAKMSAQIQNHINEKWKGRDVIAVVPLVKELVFNVSSNLFFSMNDSEELHRLHQIFETIVDGHVSMPIDLPGFTFHKALQGRAKLKKVYSSLIERRRSDLSSGLASANQDLISVLLTYKDDRGYTMTHDELLDNFLSLIESSYDSINSPMACIFKLLYANPECYEKVVQEQLGILSGKKEGEEISWKDLRSMKYTWQAIQETLRIYTQVAGIFRKAMTDIHYDGHTIPKGWQLLWATQTTHLNDKYFSEPEKFMPSRFDEEGNNVIPYSFVPFGGGRRMCPGWEFGKMEILLFVHHFVKTFSGFTPIDPNEKITGNPFPHLPANGFLIKPILRS

SEQ ID NO: 36 - protein, 493 aa, unidentified
  source 1..493: note = TOT8 protein sequence; note (original language) = TOT8蛋白序列
MDTVRELNGGSGSPGIPLSLITAAVGAIIILSLLLLRRSKRGNSSHPPGNSGLPFIGETLSFTKAFKSNTLDQFFEERVKKFGQVFKLSVIGPPTVAMCGPEGNRFVFANEEKLVHLSWSGRYAKILGGDSVSMKRGDDHRRVRAAFAGFLSPASLPVYISKMSAQIQDHINEKWKEKVVIAVVPLVKELVFNVSYNLFFSINDSEELHRLHKIFETIVEGHVSMPIDLPGFTFHRALQGRAKLKKVFSSLIERRRSDLSSGLASANQDLISVLLTYKDDRGYTMTHDELLDNFLSLLESSYDSVNSPMACIFKLLYDNPECYEKVVQEQLGILSGKKEGQEISWKDLRSMKYTWQVLQETLRLYTQVAGIFRKAMTDIHYDGHTIPKGWQLLWATQTTHLNDKYFSEPEKFMPSRFDEEGNNLIPYSFVPFGGGRRMCPGWEFGKMEILLFVHHFVKAFSGFTPIDPDEKITGNPFPHLPANGFSIKPTPRS

SEQ ID NO: 37 - protein, 493 aa, unidentified
  source 1..493: note = TOT9 protein sequence; note (original language) = TOT9蛋白序列
MDTVRELNGGSGSPGIPLSLITAAVGAIIILSLLLLRRSKRGNSSHPPGNSGLPFIGETLSFTKAFKSNTLDQFFEERVKKFGQVFKLSVIGPPTVAMCGPEGNRFVFANEEKLVHLSWSGRYAKILGGDSVSMKRGDDHRRVRAAFAGFLSPASLPVYISKMSAQIQDHINEKWKEKVVIAVVPLVKELVFNVSYNLFFSINDSEELHRLHKIFETIVEGHVSMPIDLPGFTFHRALQGRAKLKKVFSSLIERRRSDLSSGLASANQDLISVLLTYKDDRGYTMTHDELLDNFLSLLESSYDSVNSPMACIFKLLYDNPECYEKVVQEQLGILSGKKEGQEISWKDLRSMKYTWQVLQETLRLYTQVAGIFRKAMTDIHYDGHTIPKGWQLLWATQTTHLNDKYFSEPEKFMPSRFDEEGNNLIPYSFVPFGGGRRMCPGWEFGKMEILLFVHHFVKTFSGFTPIDPDEKITGNPFPHLPANGFSIKPTPRS

SEQ ID NO: 38 - protein, 507 aa, unidentified
  source 1..507: note = TOT10 protein sequence; note (original language) = TOT10蛋白序列
MVHVLQVVKMDRVSEIFNGSSGSPAGIPHSVITAGVGAIIIILLSLVLLRRSSKRGDSSHPPGNSGLPFIGETLSFTKAFKSNTLAEFFEERVKKFGNVFKISIIGPPTVVMCGNEGNRFIFANEEKLMHLSWSGRYAKILGGESVSMKRGDDHRSVRAAFAGFLSPSALPLYVAKMSAQIQNHINEKWKGRDVIAVVPLVKELVFNVSSNLFFSMNDSEELHLLHQIFETIVDGHVSMPIDLPGFTFHKALQGRAKLKKVYSSLIERRRSDLSSGLASANQDLISVLLTYKDDRGYTMTHDELLDNFLSLIESSYDSINSPMACIFKLLYANPECYEKVVQEQLGILSGKKEGEEISWKDLRSMKYTWQAIQETLRIYTQVAGIFRKAMTDIHYDGHTIPKGWQLLWATQTTHLNDKYFSEPEKFMPSRFDEEGNNVIPYSFVPFGGGRRMCPGWEFGKMEILLFVHHFVKTFSGFTPIDPNEKITGNPFPHLPANGFLIKPILRS

SEQ ID NO: 39 - protein, 493 aa, unidentified
  source 1..493: note = TOT11 protein sequence; note (original language) = TOT11蛋白序列
MDTVRELNGGSGSPGIPLSLITAAVGAIIILSLLLLRRSKRGNSSHPPGNSGLPFIGETLSFTKAFKSNTLDQFFEERVKKFGQVFKLSVIGPPTVAMCGPEGNRFVFANEEKLVHLSWSGRYAKILGGDSVSMKRGDDHRSVRAAFAGFLSPASLPVYISKMSAQIQDHINEKWKGKDVIAVVPLVKELVFNVSYNLFFSLNDSEELHRLHKIFETIVEGHVSMPIDLPGFTFHRALQGRAKLKKVFSSLIERRRSDLSSGLASANQDLISVLLTYKDDRGYTMTHDELLDNFLSLLEASYDSVNSPMACIFKLLYDNPECYEKVVQEQLGILSGKKEGQEISWKDLRSMKYTWQVLQETLRLYTQVAGIFRKAMTDIHYDGHTIPKGWQLLWATQTTHLNDKYFSEPEKFMPSRFDEEGNNLIPYSFVPFGGGRRMCPGWEFGKMEILLFVHHFVKTFSGFTPIDPDEKITGNPFPHLPANGFSIKPTPRS

SEQ ID NO: 40 - protein, 498 aa, unidentified
  source 1..498: note = TOT12 protein sequence; note (original language) = TOT12蛋白序列
MDRVREIFNGSSGSPAGIPHSVITAGVGAIIIILLSLLLLRRSSKRGDSSHPPGNSGLPFIGETLSFTKAFKSNTLAEFFEERVKKFGNVFKISIIGPPTVVMCGNEGNRFIFANEEKLMHLSWSGRYAKILGGESVSMKRGDDHRSVRAAFAGFLSSASLPVYISKMSAQIQDHINEKWKGKDVIAVVPLVKELVFNVSYNLFFSINDSEELHRLHKIFETIVEGHLSMPIDLPGFTFHRALQGRAKLKKVFSSLIERRRSDLSSGLASANQDLISVLLTYKDDRGYTMTHDELLDNFLSLLEGSYDSINSPMACIFKLLYDNPECYEKVVQEQLGILSGKKEGQEISWKDLRSMKYTWQVLQETLRLYTQVAGIFRKAMTDIHYDGHTIPKGWQLLWANQTTHLNDKYFSEPEKFMPSRFDEEGNNMIPYSFVPFGGGRRMCPGWEFGKMEILLFVHHFVKTFSGFTPIDPNEKITGNPFPHLPANGFLIKPILRS

SEQ ID NO: 41 - protein, 498 aa, unidentified
  source 1..498: note = TOT13 protein sequence; note (original language) = TOT13蛋白序列
MDRVSEIFNGSSGSPAGIPHSVITAGVGAIIIILLSLVLLRRSSKRGDSSHPPGNSGLPFIGETLSFTKAFKSNTLAEFFEERVKKFGNVFKISIIGPPTVVMCGNEGNRFIFANEEKLMHLSWSGRYAKILGGESVSMKRGDDHRSVRAAFAGFLSPSALPLYVAKMSAQIQNHINEKWKGRDVIAVVPLVKELVFNVSSNLFFSMNDSEELHLLHQIFETIVDGHVSMPIDLPGFTFHKALQGRAKLKKVYSSLIERRRSDLSSGLASANQDLISVLLTYKDDRGYTMTHDELLDNFLSLIESSYDSINSPMACIFKLLYANPECYEKVVQEQLGILSGKKEGEEISWKDLRSMKYTWQAIQETLRIYTQVAGIFRKAMTDIHYDGHTIPKGWQLLWATQTTHLNDKYFSEPEKFMPSRFDEEGNNVIPYSFVPFGGGRRMCPGWEFGKMEILLFVHHFVKTFSGFTPIDPNEKITGNPFPHLPANGFLIKPILRS

SEQ ID NO: 42 - protein, 507 aa, unidentified
  source 1..507: note = TOT14 protein sequence; note (original language) = TOT14蛋白序列
MVHVLQVVKMDRVREIFNGSSGSPAGIPHSVITAGVGAIIIILLSLLLLRRSSKRGDSSHPPGNSGLPFIGETLSFTKAFKSNTLAEFFEERVKKFGNVFKISIIGPPTVVMCGNEGNRFIFANEEKLMHLSWSGRYAKILGGESVSMKRGDDHRSVRAAFAGFLSPASLPIYISKMSAQIQDHINKKWKGKDVIAVVPLVKELVFNVSYNLFFSINDSEELHRLHKIFETIVEGHVSMPIDLPGFTFHRALQGRAKLKKVYSSLIERRRSDLSSGLASANQDLISVLLTYKDDRGYRMTHDELLDNFLSLLESSYDSVNSPMACILKLLYANPECYEKVVQEQLGILSGKKEGEEISWKDLRSMKYTWQVLQETLRLYTQVAGIFRKAMTDIHYDGHTIPKGWQLLWATQTTHLNDKYFSEPEKFMPSRFDEEGNNVIPYSFVPFGGGRRMCPGWEFGKMEILLFVHHFVKTFSGFTPIDPNEKITGNPFPHLPANGFLIKPILRS

SEQ ID NO: 43 - protein, 507 aa, unidentified
  source 1..507: note = TOT15 protein sequence; note (original language) = TOT15蛋白序列
MVHVLQVVKMDRVREIFNGSSGSPAGIPHSVITAGVGAIIIILLSLLLLRRSSKRGDSSHPPGNSGLPFIGETLSFTKAFKSNTLAEFFEERVKKFGNVFKISIIGPPTVVMCGNEGNRFIFANEEKLMHLSWSGRYAKILGGESVSMKRGDDHRSVRAAFAGFLSPSALPLYVAKMSAQIQNHINEKWKGRDVIAVVPLVKELVFNVSSNLFFSMNDSEELHRLHQIFETIVDGHVSMPIDLPGFTFHKALQGRAKLKKVYSSLIERRRSDLSSGLASANQDLISVLLTYKDDRGYRMTHDELLDNFLSLLESSYDSVNSPMACILKLLYANPECYEKVVQEQLGILSGKKEGEEISWKDLRSMKYTWQVLQETLRLYTQVAGIFRKAMTDIHYDGHTIPKGWQLLWATQTTHLNDKYFSEPEKFMPSRFDEEGNNVIPYSFVPFGGGRRMCPGWEFGKMEILLFVHHFVKTFSGFTPIDPNEKITGNPFPHLPANGFLIKPILRS

SEQ ID NO: 44 - protein, 498 aa, unidentified
  source 1..498: note = TOT16 protein sequence; note (original language) = TOT16蛋白序列
MDRVREIFNGSSGSPAGIPHSVITAGVGAIIIILLSLLLLRRSSKRGDSSHPPGNSGLPFIGETLSFTKAFKSNTLAEFFEERVKKFGNVFKISIIGPPTVVMCGNEGNRFIFANEEKLMHLSWSGRYAKILGGESVSMKRGDDHRSVRAAFAGFLSPASLPIYISKMSAQIQDHINKKWKGKDVIAVVPLVKELVFNVSYNLFFSINDSEELHRLHKIFETIVEGHVSMPIDLPGFTFHRALQGRAKLKKVYSSLIERRRSDLSSGLASANQDLISVLLTYKDDRGYRMTHDELLDNFLSLLESSYDSVNSPMACILKLLYANPECYEKVVQEQLGILSGKKEGEEISWKDLRSMKYTWQVLQETLRLYTQVAGIFRKAMTDIHYDGHTIPKGWQLLWATQTTHLNDKYFSEPEKFMPSRFDEEGNNVIPYSFVPFGGGRRMCPGWEFGKMEILLFVHHFVKTFSGFTPIDPNEKITGNPFPHLPANGFLIKPILRS

SEQ ID NO: 45 - protein, 498 aa, unidentified
  source 1..498: note = TOT17 protein sequence; note (original language) = TOT17蛋白序列
MDRVREIFNGSSGSPAGIPHSVITAGVGAIIIILLSLLLLRRSSKRGDSSHPPGNSGLPFIGETLSFTKAFKSNTLAEFFEERVKKFGNVFKISIIGPPTVVMCGNEGNRFIFANEEKLMHLSWSGRYAKILGGESVSMKRGDDHRSVRAAFAGFLSPSALPLYVAKMSAQIQNHINEKWKGRDVIAVVPLVKELVFNVSSNLFFSMNDSEELHRLHQIFETIVDGHVSMPIDLPGFTFHKALQGRAKLKKVYSSLIERRRSDLSSGLASANQDLISVLLTYKDDRGYRMTHDELLDNFLSLLESSYDSVNSPMACILKLLYANPECYEKVVQEQLGILSGKKEGEEISWKDLRSMKYTWQVLQETLRLYTQVAGIFRKAMTDIHYDGHTIPKGWQLLWATQTTHLNDKYFSEPEKFMPSRFDEEGNNVIPYSFVPFGGGRRMCPGWEFGKMEILLFVHHFVKTFSGFTPIDPNEKITGNPFPHLPANGFLIKPILRS

SEQ ID NO: 46 - protein, 507 aa, unidentified
  source 1..507: note = TOT18 protein sequence; note (original language) = TOT18蛋白序列
MVHVLQVVKMDRVSEIFNGSSGSPAGIPHSVITAGVGAIIIILLSLLLLRRSSKRGDSSHPPGNSGLPFIGETLSFTKAFKSNTLAEFFEERVKKFGNVFKISIIGPPTVVMCGNEGNRFIFANEEKLMHLSWSGRYAKILGGESVSMKRGDDHRSVRAAFAGFLSPSALPLYVAKMSAQIQNHINEKWKGRDVIAVVPLVKELVFNVSSNLFFSMNDSEELHRLHQIFETIVDGHVSMPIDLPGFTFHKALQGRAKLKKVYSSLIERRRSDLSSGLASANQDLISVLLTYKDDRGYTMTHDELLDNFLSLIESSYDSINSPMACIFKLLYANPECYEKVVQEQLGILSGKKEGEEISWKDLRSMKYTWQAIQETLRIYTQVAGIFRKAMTDIHYDGHTIPKGWQLLWATQTTHLNDKYFSEPEKFMPSRFDEEGNNVIPYSFVPFGGGRRMCPGWEFGKMEILLFVHHFVKTFSGFTPIDPNEKITGNPFPHLPANGFLIKPILRS

SEQ ID NO: 47 - protein, 497 aa, unidentified
  source 1..497: note = TOT19 protein sequence; note (original language) = TOT19蛋白序列
MDVFYPLKSAVTKFNECFPAILFIVLSAVAGIVLPLLLFLRSKRRSSVGLPPGKLGYPFIGESLLFLKALRSNTVEQFLDERVKKFGNVFKTSLIGHPTVVLCGPAGNRLILANEEKLVQMSWPKSSMKLMGEKSITAKRGEGHMIIRSALQGFFSPGALQKYIGQMSKTIENHINEKWKGNDQVSVVALVGDLVFDISACLFFNINEKHERERLFELLEIIAVGVLAVPVDLPGFAYRRALQARSKLNAILSGLIEKRKMDLSSGLASSNQDLLSVFLTFKDDRGNPLSDEEILDNFSGLLHGSYDTTVSAMACVFKLLSSNPECYEKVVQEQLGILSGKKEGQEISWKDLRSMKYTWQVLQETLRLYTQVAGIFRKAMTDIHYDGHTIPKGWQLLWATQTTHLNDKYFSEPEKFMPSRFDEEGNNVIPYSFVPFGGGRRMCPGWEFGKMEILLFVHHFVKAFSGFTPIDPDEKITGNPFPHLPANGFLIKPILRS

SEQ ID NO: 48 - protein, 498 aa, unidentified
  source 1..498: note = TOT20 protein sequence; note (original language) = TOT20蛋白序列
MDRVSEIFNGSSGSPAGIPHSVITAGVGAIIIILLSLLLLRRSSKRGDSSHPPGNSGLPFIGETLSFTKAFKSNTLAEFFEERVKKFGNVFKISIIGPPTVVMCGNEGNRFIFANEEKLMHLSWSGRYAKILGGESVSMKRGDDHRSVRAAFAGFLSPSALPLYVAKMSAQIQNHINEKWKGRDVIAVVPLVKELVFNVSSNLFFSMNDSEELHRLHQIFETIVDGHVSMPIDLPGFTFHKALQGRAKLKKVYSSLIERRRSDLSSGLASANQDLISVLLTYKDDRGYTMTHDELLDNFLSLIESSYDSINSPMACIFKLLYANPECYEKVVQEQLGILSGKKEGEEISWKDLRSMKYTWQAIQETLRIYTQVAGIFRKAMTDIHYDGHTIPKGWQLLWATQTTHLNDKYFSEPEKFMPSRFDEEGNNVIPYSFVPFGGGRRMCPGWEFGKMEILLFVHHFVKTFSGFTPIDPNEKITGNPFPHLPANGFLIKPILRS

SEQ ID NO: 49 - protein, 507 aa, unidentified
  source 1..507: note = TOT21 protein sequence; note (original language) = TOT21蛋白序列
MVHVLQVVKMDRVNEIFNGSSGSPAGIPHSVITAGVGAIIIILLSLLLLRRSSKRGDSAHPPGNSGLPFIGETLSFTKAFKSNTLAEFFEERVKKFGNVFKISIIGPPTVVMCGNEGNRFIFANEEKLMHLSWSGRYAKILGGESVSMKRGDDHRSVRAAFAGFLSSASLPVYISKMSAQIQDHINEKWKGKDVIAVVPLVKELVFNVSYNLFFSINDSEELHRLHKIFETIVEGHVSMPIDLPGFTFHRALQGREKLKKVFSSLIERRRSDLSSGLASANQDLISVLLTYKDDRGYTMTHDELLDNFLSLLESSYDSVNSPMACIFKLLYDNPECYEKVVQEQLGILSGKKEGQEISWKDLRSMKYTWQVLQETLRLYTQVAGIFRKAMTDIHYDGHTIPKGWQLLWATQTTHLNDKYFSEPEKFMPSRFGEEGNNLIPYSFVPFGGGRRMCPGWEFGKMEILLFVHHFVKTFSGFTPIDPDEKITGNPFPHLPANGFSIKPTPRS

SEQ ID NO: 50 - protein, 498 aa, unidentified
  source 1..498: note = TOT22 protein sequence; note (original language) = TOT22蛋白序列
MDRVNEIFNGSSGSPAGIPHSVITAGVGAIIIILLSLLLLRRSSKRGDSAHPPGNSGLPFIGETLSFTKAFKSNTLAEFFEERVKKFGNVFKISIIGPPTVVMCGNEGNRFIFANEEKLMHLSWSGRYAKILGGESVSMKRGDDHRSVRAAFAGFLSSASLPVYISKMSAQIQDHINEKWKGKDVIAVVPLVKELVFNVSYNLFFSINDSEELHRLHKIFETIVEGHVSMPIDLPGFTFHRALQGREKLKKVFSSLIERRRSDLSSGLASANQDLISVLLTYKDDRGYTMTHDELLDNFLSLLESSYDSVNSPMACIFKLLYDNPECYEKVVQEQLGILSGKKEGQEISWKDLRSMKYTWQVLQETLRLYTQVAGIFRKAMTDIHYDGHTIPKGWQLLWATQTTHLNDKYFSEPEKFMPSRFGEEGNNLIPYSFVPFGGGRRMCPGWEFGKMEILLFVHHFVKTFSGFTPIDPDEKITGNPFPHLPANGFSIKPTPRS

SEQ ID NO: 51 - protein, 507 aa, unidentified
  source 1..507: note = TOT23 protein sequence; note (original language) = TOT23蛋白序列
MVHVLQVVKMDRVSEIFNGSSGSPAGIPHSVITAGVGAIIIILLSLVLLRRSSKRGDSSHPPGNSGLPFIGETLSFTKAFKSNTLAEFFEERVKKFGNVFKISIIGPPTVVMCGNEGNRFIFANEEKLMHLSWSGRYAKILGGESVSMKRGDDHRSVRAAFAGFLSPSALPLYVAKMSAQIQNHINEKWKGRDVIAVVPLVKELVFNVSSNLFFGMNDSEELHRLHQIFETIVDGHVSMPIDLPGFTFHKALQGRAKLKKVYSSLIERRRSDLSSGLASANQDLISVLLTYKDDRGYTMTHVELLDNFLSLIESSYDSINSPMACIFKLLYANPECYEKVVQEQLGILSGKKKGEEISWKDLRSMKYTWQAIQETLRIYTQVAGIFRKAMTDIHYDGHTIPKGWQLLWATQTTHLNDKYFSEPEKFMPSRFDEEGNNVIPYSFVPFGGGRRMCPGWEFGKMEILLFVHHFVKTFSGFTPIDPNEKITGNPFPHLPANGFLIKPILRS

SEQ ID NO: 52 - protein, 510 aa, unidentified
  source 1..510: note = TOT24 protein sequence; note (original language) = TOT24蛋白序列
MDSLHRVIKISAIFNGDTKLHWSSPAVFSVAFTAVAGILLLLLLLRSKRRHSSLNQYNLPRGNSGLPFVGETISFLRAFRGNRIQQFFDERAKKFGNVFRISITGPPTAVLCGSEGNRFILSNEEKLVRVDMSGAFSKLAGRDSVMMRTGEEHRTIRAAMAGFLAPTALPIYVGKMSAQIQNHIDEKWKGKDVVTVVSLVKELVFGVSASMFYDINDGVEQHRLHEIYQTMVAGHFSFPLDFPGFSFHRAVQGRQKLKKIFSSLIEKRRSDLRSGLASSNQDLLSVLLTYKNEKGNGLTQGELTDNFITMLEASYDNPVSAISCILKFLYSHPEVYEKVVQEQLGILSNKEEGDEISWKDVKAMKYTWQAVQETLRMISPVIGILRKAMTDIHYDGYTIPKGWQLLWTGCSTHLKDAYFNEADEFMPSRFDEEGKNVVPYSFVPFGGGRRMCPGWEFSKLAILLFVHHFVKTFSSYTPLDPDEKILGNPFPLLPVNGLSIKLTARSEIKN

SEQ ID NO: 53 - DNA, 1524 bp, unidentified
  source 1..1524: mol_type = other DNA; note = TOT1 reading frame nucleotide sequence; note (original language) = TOT1读码框核苷酸序列
atggttcatgtgttgcaggtagtgaaaatggatagagttagagaaatatttaatggaagttcaggttctccagctggtattccccacagtgtgatcacagccggtgtgggtgccataataataattcttctgtcactactgctcctccgccgttctagtaaacggggcgactcctctcatcctcctgggaattcaggccttccattcattggagagacattatcattcaccaaggcttttaaatcgaacacgctggccgaattttttgaggagagggtgaagaaattcgggaatgtatttaagatttcaataatcgggcctcccacagtggtaatgtgcggcaatgagggaaaccggtttattttcgccaacgaggagaagcttgtccacttgtcgtggtctggtcgatatgcgaaaatcctgggtggagattccgtttccatgaagaggggagatgatcatcgcagtgtacgtgccgcattcgcagggtttttgagccctgcatcgctgcctatttacataagtaaaatgagtgcacagatccaagatcatatcaaccaaaaatggaaaggaaaagatgtaattgctgtagttcctctggtaaaggagctcgtcttcaacgtttcctacaacttgtttttcagcataaatgatagcgaggaactgcatcgattgcataagattttcgaaactattgtggagggacatgtttccatgccgatagaccttcccggattcacctttcatagagcacttcagggaagggcgaagctcaagaaagttttctcttctttaatagaaaggagaagaagcgatctgagctccggattggcatctgctaatcaggatctcatctctgttttactcacctacaaagatgatagggggtatacaatgacccacgacgagctcctcgacaactttctttcccttcttgaatcctcctatgattccgtcaattcaccaatggcctgcatttttaagcttttgtatgccaatccagaatgctatgaaaaagtagttcaagagcaattggggatactttctggtaagaaggaaggacaagaaatctcgtggaaggatctgagatccatgaaatacacatggcaagtacttcaggaaacgctacgactgtatactcaagttgctggaatatttcgcaaagccatgactgtcattcattatgatggtcacaccattcccaaagggtggcaacttctttgggcaacccaaactacacatctgaacgacaaatatttcagtgagccggaaaaattcatgccttccagattcgatgaagaaggaaacaatgtgattccttactcattcgtaccatttggaggagggcggcggatgtgtccaggttgggaattcggaaagatggagatcttactcttcgtccatcactttgttaaagcgttcagtggctttaccccaatcgatccggacgaaaaaattactgggaatccatttcctcatctccctgccaatggattttcaataaaacctactcccagatcctaa

SEQ ID NO: 54 - DNA, 1524 bp, unidentified
  source 1..1524: mol_type = other DNA; note = TOT2 reading frame nucleotide sequence; note (original language) = TOT2读码框核苷酸序列
atggttcatgtgttgcaggtagtgaaaatggatagagttagtgaaatatttaatggaagttcaggttctccagctggtattccccacagtgtgatcacagccggtgtgggtgccataataataattcttctgtcactagtgctcctccgccgttctagtaaacggggcgactcctctcatcctcctgggaattcaggccttccattcattggggagacattatcattcaccaaggcttttaaatcgaacacgctggccgaattttttgaggagagggtgaagaaattcgggaatgtatttaagatttcaataatcgggcctcccacagtggtaatgtgcggcaatgagggaaaccggtttattttcgccaacgaggagaagctgatgcacctgtcgtggtccggtcggtatgcgaaaatccttggtggggaatccgtttccatgaagaggggagatgatcatcgcagtgtacgtgccgcattcgcagggtttttgagcccttcggcgctgcctctttacgtagctaaaatgagtgcgcagatccaaaatcatatcaacgagaaatggaaaggaagagatgtaattgctgtagttcctttggtaaaagagctggtcttcaacgtttcctccaacttgtttttcagcatgaatgatagcgaggaattgcatcgattgcatcaaattttcgaaactattgtagatggacatgtttccatgccgatagaccttcccggattcacctttcataaagcacttcagggaagggcgaagctcaagaaagtttactcttctttaatagaaaggagaagaagcgatctgagctccggattggcatctgctaatcaggatctcatctctgttttactcacctacaaagatgatagggggtatacaatgacccacgacgagctcctcgacaattttctttcccttattgaatcctcctatgattccatcaattcaccaatggcctgcatttttaagcttttgtatgccaatccagaatgctatgaaaaagtagttcaagagcaattggggatactttctggtaagaaggaaggagaagaaatctcatggaaggatctgagatccatgaaatacacatggcaagcaattcaggaaacgctacgaatttatactcaagttgcaggaatatttcgcaaagccatgactgacattcattatgatggtcacaccattcccaaagggtggcaacttctttgggcaacccaaactacacatctgaacgacaaatatttcagtgagcctgaaaaattcatgccttccagattcgatgaagaaggaaacaatgtgattccttactcattcgtaccatttggaggagggcggcggatgtgtccaggttgggaattcggaaagatggagatcttactctttgtccatcactttgttaaaacgttcagtggctttaccccaattgatccgaacgaaaaaattactgggaatccttttcctcatctccctgccaatggatttctaataaaacctattctcagatcctaa

SEQ ID NO: 55 - DNA, 1524 bp, unidentified
  source 1..1524: mol_type = other DNA; note = TOT3 reading frame nucleotide sequence; note (original language) = TOT3读码框核苷酸序列
atggttcatgtgttgcacgtagtgaaaatggatagagttagagaaatatttaatggaagttcaggttctccagctggtattccccacagtgtgatcacagccggtgtgggtgccataataataattcttctgtcactactgctcctccgccgttctagtaaacggggcgactcctctcatcctcctgggaattcaggccttccattcattggggagacattatcattcaccaaggcttttaaatcgaacacgctggccgaattttttgaggagagggtgaagaaattcgggaatgtatttaagatttcaataatcgggcctcccacagtggtaatgtgcggcaatgagggaaaccggtttattttcgccaacgaggagaagctgatgcacctgtcgtggtccggtcgatatgcgaaaatccttggtggggaatccgtttccatgaagaggggagatgatcatcgcagtgtacgtgccgcattcgcagggtttttgagctctgcatcgctgcctgtttacataagtaaaatgagtgcacagatccaagatcatatcaacgaaaaatggaaaggaaaagatgtaattgctgtagttcctctggtaaaggagctcgtcttcaacgtttcctacaacttgtttttcagcataaatgatagcgaggaactgcatcgattgcataagattttcgaaactattgtggagggacatctttccatgccgatagaccttcccggattcacctttcatagagcacttcagggaagggcgaagctcaagaaagttttctcttctttaatagaaaggagaagaagcgatctgagctccggattggcatctgctaatcaggatctcatttctgttttactcacctacaaagatgatagggggtatacaatgacccacgacgagctcctcgacaactttctttcccttcttgaaggctcctatgattccatcaattcaccaatggcctgcatttttaagcttttgtatgacaatccagaatgctatgaaaaagtagttcaagagcaattggggatactttctggtaagaaggaaggacaagaaatctcgtggaaggatctgagatccatgaaatacacatggcaagtacttcaggaaacgctacgactgtatactcaagttgctggaatatttcgcaaagccatgactgacattcattatgatggtcacaccattcccaaagggtggcaacttctttgggcaaaccaaactacacatctgaacgacaaatatttcagtgagcctgaaaaattcatgccttccagattcgatgaagaaggaaacaatatgattccttactcattcgtaccatttggaggagggcggcggatgtgtccaggttgggaattcggaaagatggagatcttactctttgtccatcactttgttaaaacgttcagtggctttaccccaattgatccgaacgaaaaaattactgggaatccttttcctcatctccctgccaatggatttctaataaaacctattctcagatcctaa

SEQ ID NO: 56 - DNA, 1524 bp, unidentified
  source 1..1524: mol_type = other DNA; note = TOT4 reading frame nucleotide sequence; note (original language) = TOT4读码框核苷酸序列
atggttcatgtgttgcaggtagtgaaaatggatagagttagtgaaatatttaatggaagttcaggttctccagctggtattccccacagtgtgatcacagccggtgtgggtgccataataataattcttctgtcactagtgctcctccgccgttctagtaaacggggcgactcctctcatcctcctgggaattcaggccttccattcattggggagacattatcattcaccaaggcttttaaatcgaacacgctggccgaattttttgaggagagggtgaagaaattcgggaatgtatttaagatttcaataatcgggcctcccacagtggtaatgtgcggcaatgagggaaaccggtttattttcgccaacgaggagaagctgatgcacctgtcgtggtccggtcggtatgcgaaaatccttggtggggaatccgtttccatgaagaggggagatgatcatcgcagtgtacgtgccgcattcgcagggtttttgagcccttcggcgctgcctctttacgtagctaaaatgagtgcgcagatccaaaatcatatcaacgagaaatggaaaggaagagatgtaattgctgtagttcctttggtaaaagagctggtcttcaacgtttcctccaacttgtttttcagcatgaatgatagcgaggaattgcatcgattgcatcaaattttcgaaactattgtagatggacatgtttccatgccgatagaccttcccggattcacctttcataaagcacttcagggaagggcgaagctcaagaaagtttactcttctttaatagaaaggagaagaagcgatctgagctccggattggcatctgctaatcaggatctcatctctgttttactcacctacaaagatgatagggggtatacaatgacccacgacgagctcctcgacaattttctttcccttattgaatcctcctatgattccgtcaattcaccaatggcctgcatttttaagcttttgtatgccaatccagaatgctatgaaaaagtagttcaagagcaattggggatactttctggtaagaaggaaggacaagaaatctcgtggaaggatctgagatccatgaaatacacatggcaagtacttcaggaaacgctacgactgtatactcaagttgctggaatatttcgcaaagccatgactgtcattcattatgatggtcacaccattcccaaagggtggcaacttctttgggcaacccaaactacacatctgaacgacaaatatttcagtgagccgcaaaaattcatgccttccagattcgatgaagaaggaaacaatgtgattccttactcattcgtaccatttggaggagggcggcggatgtgtccaggttgggaattcggaaagatggagatcttactcttcgtccatcactttgttaaagcgttcagtggctttaccccaatcgatccggacgaaaaaattactgggaatccttttcctcatctccctgccaatggatttctaataaaacctattctcagatcctaa

SEQ ID NO: 57 - DNA, 1482 bp, unidentified
  source 1..1482: mol_type = other DNA; note = TOT5 reading frame nucleotide sequence; note (original language) = TOT5读码框核苷酸序列
atggatacagttagagaattgaatggaggatcaggttcctctggtattcccctcagtctgatcaccgccgctgtgggtgccataataattctgtcactactgctcctccgccgttctaaacggggcaactcatctcatcctcctgggaattcagggcttccattcattggggagacattatcattcaccaaggcttttaaatcgaacacgctggaccaattttttgaggagagggtgaagaaattcgggcaagtctttaagctttccgtaatcgggcctcccacagtggcaatgtgcggccctgagggaaaccggtttgttttcgccaacgaggagaagcttgtccacttgtcgtggtctggtcgatatgcgaaaatcctgggtggagattccgtttccatgaagaggggagatgatcatcgcagtgtacgtgccgcattcgcagggtttttgagccctgcatcgctgcctgtttacataagtaaaatgagtgcacagatccaagatcatatcaacgaaaaatggaaaggaaaagatgtaattgctgtagttcctctggtaaaggagctcgtcttcaacgtttcctacaacttgtttttcagcataaatgatagcgaggaactgcatcgattgcataagattttcgaaactattgtggagggacatgtttccatgccgatagaccttcccggattcacctttcatagagcacttcagggaagggcgaagctcaagaaagttttctcttctttaatagaaaggagaagaagcgatcttagctccggattggcatctgctaatcaggatctcatttctgttttactcacctacaaagatgatagggggtatacaatgacccacgacgagctcctcgacaactttctttcccttcttgaagcctcctatgattccgtcaattcaccaatggcctgcatttttaagcttttgtatgccaatccagaatgctatgaaaaagtagttcaagagcaattggggatactttctggtaagaaggaaggacaagaaatctcgtggaaggatctgagatccatgaaatacacatggcaagtacttcaggaaacgctacgactgtatactcaagttgctggaatatttcgcaaagccatgactgacattcattataatggtcataccattcccaaagggtggcaacttctttgggcaacccaaactacacatctgaacgacaaatatttcagtgagccggaaaaattcatgccttccagattcgatgaagaaggaaacaatgtgattccttactcattcgtaccatttggaggagggcggcggatgtgtccaggttgggaattcggaaagatggagatcttactcttcgtccatcactttgttaaagcgttcagtggctttaccccaatcgatccggacgaaaaaattactgggaatccatttcctcatctccctgccaatggattttcaataaaacctactcccagatcctaa

SEQ ID NO: 58 - DNA, 1524 bp, unidentified
  source 1..1524: mol_type = other DNA; note = TOT6 reading frame nucleotide sequence; note (original language) = TOT6读码框核苷酸序列
atggttcatgtgttgcaggtagtgaaaatggatagagttagtgaaatatttaatggaagttcaggttctccagctggtattccccacagtgtgatcacagccggtgtgggtgccataataataattcttctgtcactagtgctcctccgccgttctagtaaacggggcgactcctctcatcctcctgggaattcaggccttccattcattggggagacattatcattcaccaaggcttttaaatcgaacacgctggccgaattttttgaggagagggtgaagaaattcgggaatgtatttaagatttcaataatcgggcctcccacagtggtaatgtgcggcaatgagggaaaccggtttattttcgccaacgaggagaagctgatgcacctgtcgtggtccggtcgatatgcgaaaatccttggtggggaatccgtttccatgaagaggggagatgatcatcgcagtgtacgtgccgcattcgcagggtttttgagcccttcggcgctgcctctttacgtagctaaaatgagtgcgcagatccaaaatcatatcaacgagaaatggaaaggaagagatgtaattgctgtagttcctttggtaaaagagctggtcttcaacgtttcctccaacttgtttttcggcatgaatgatagcgaggaactgcatcgattgcatcaaattttcgaaactattgtagatggacatgtttccatgccgatagaccttcccggattcacctttcataaagcacttcagggaagggcgaagctcaagaaagtttactcttctttaatagaaaggagaagaagcgatctgagctccggattggcatctgctaatcaggatctcatctctgttttactcacctacaaagatgatagggggtatacaatgacccacgtcgagctcctcgacaattttctttcccttattgaatcctcctatgattccatcaattcaccaatggcctgcatttttaagcttttgtatgccaatccagaatgctatgaaaaagtagttcaagagcaattggggatactctctggtaagaaggaaggagaagaaatctcatggaaggatctgagatccatgaaatacacatggcaagcaattcaggaaacgctacgaatttatactcaagttgcaggaatatttcgcaaagccatgactgacattcattatgatggtcacaccattcccaaagggtggcaacttctttgggcaacccaaactacacatctgaacgacaaatatttcagtgagcctgaaaaattcatgccttccagattcgatgaagaaggaaacaatgtgattccttactcattcgtaccatttggaggagggcggcggatgtgtccaggttgggaattcggaaagatggagatcttactctttgtccatcactttgttaaaacgttcagtggctttaccccaattgatccgaacgaaaaaattactgggaatccttttcctcatctccctgccaatggatttctaataaaacctattctcagatcctaa

SEQ ID NO: 59 - DNA, 1524 bp, unidentified
  source 1..1524: mol_type = other DNA; note = TOT7 reading frame nucleotide sequence; note (original language) = TOT7读码框核苷酸序列
atggttcatgtgttgcaggtagtgaaaatgtatagagttagtgaaatatttaatggaagttcaggttctccagctggtattccccacagtgtgatcacagccggtgtgggtgccataataataattcttctgtcactagtgctcctccgccgttctagtaaacggggcgactcctctcatcctcctgggaattcaggccttccattcattggggagacattatcattcaccaaggcttttaaatcgaacacgctggccgaattttttgaggagagggtgaagaaattcgggaatgtatttaagatttcaataatcgggcctcccacagtggtaatgtgcggcaatgagggaaaccggtttattttcgccaacgaggagaagctgatgcacctgtcgtggtccggtcggtatgcgaaaatccttggtggggaatccgtttccatgaagaggggagatgatcatcgcagtgtacgtgccgcattcgcagggtttttgagcccttcggcgctgcctctttacgtagctaaaatgagtgcgcagatccaaaatcatatcaacgagaaatggaaaggaagagatgtaattgctgtagttcctttggtaaaagagctggtcttcaacgtttcctccaacttgtttttcagcatgaatgatagcgaggaattgcatcgattgcatcaaattttcgaaactattgtagatggacatgtttccatgccgatagaccttcccggattcacctttcataaagcacttcagggaagggcgaagctcaagaaagtttactcttctttaatagaaaggagaagaagcgatctgagctccggattggcatctgctaatcaggatctcatctctgttttactcacctacaaagatgatagggggtatacaatgacccacgacgagctcctcgacaattttctttcccttattgaatcctcctatgattccatcaattcaccaatggcctgcatttttaagcttttgtatgccaatccagaatgctatgaaaaagtagttcaagagcaattggggatactttctggtaagaaggaaggagaagaaatctcatggaaggatctgagatccatgaaatacacatggcaagcaattcaggaaacgctacgaatttatactcaagttgcaggaatatttcgcaaagccatgactgacattcattatgatggtcacaccattcccaaagggtggcaacttctttgggcaacccaaactacacatctgaacgacaaatatttcagtgagcctgaaaaattcatgccttccagattcgatgaagaaggaaacaatgtgattccttactcattcgtaccatttggaggagggcggcggatgtgtccaggttgggaattcggaaagatggagatcttactctttgtccatcactttgttaaaacgttcagtggctttaccccaattgatccgaacgaaaaaattactgggaatccttttcctcatctccctgccaatggatttctaataaaacctattctcagatcctaa

SEQ ID NO: 60 - DNA, 1482 bp, unidentified
  source 1..1482: mol_type = other DNA; note = TOT8 reading frame nucleotide sequence; note (original language) = TOT8读码框核苷酸序列
atggatacagttagagaattgaatggaggatcaggttcccctggtattcccctcagtctgatcaccgccgctgtgggtgccataataattctgtcactactgctcctccgccgttctaaacggggcaactcatctcatcctcctgggaattcagggcttccattcattggggagacattatcattcaccaaggcttttaaatcgaacacgctggaccaattttttgaggagagggtgaagaaattcgggcaagtctttaagctttccgtaatcgggcctcccacagtggcaatgtgcggccctgagggaaaccggtttgttttcgccaacgaggagaagcttgtccacttgtcgtggtctggtcgatatgcgaaaatcctgggtggagattccgtttccatgaagaggggagatgatcatcgcagagtacgtgccgcattcgcagggtttttgagccctgcatcactgcctgtttacataagtaaaatgagtgcacagatccaagatcatatcaacgaaaaatggaaagaaaaagttgtaattgctgtagttcctctggtaaaggagctcgtcttcaacgtttcctacaacttgtttttcagcataaatgatagcgaggaactgcatcgattgcataagattttcgaaactattgtggagggacatgtttccatgccgatagaccttcccggattcacctttcatagagcacttcagggaagggcgaagctcaagaaagttttctcttctttaatagaaaggagaagaagcgatctgagctccggattggcatctgctaatcaggatctcatctctgttttactcacctacaaagatgatagggggtatacaatgacccacgacgagctcctcgacaactttctttcccttcttgaatcctcctatgattccgtcaattcaccaatggcctgcatttttaagcttttgtatgacaatccagaatgctatgaaaaagtagttcaagagcaattggggatactttctggtaagaaggaaggacaagaaatctcgtggaaggatctgagatccatgaaatacacatggcaagtacttcaggaaacgctacgactgtatactcaagttgctggaatatttcgcaaagccatgactgacattcattatgatggtcacaccattcccaaagggtggcaacttctttgggcaacccaaactacacatctgaacgacaaatatttcagtgagccggaaaagttcatgccttccagattcgatgaagaaggaaacaatttgattccttactcattcgtaccatttggaggagggcggcggatgtgtccaggttgggaattcggaaagatggagatcttactcttcgtccatcactttgttaaagcgttcagtggctttaccccaatcgatccggacgaaaaaattactgggaatccatttcctcatctccctgccaatggattttcaataaaacctactcccagatcctaa

SEQ ID NO: 61 - DNA, 1482 bp, unidentified
  source 1..1482: mol_type = other DNA; note = TOT9 reading frame nucleotide sequence; note (original language) = TOT9读码框核苷酸序列
atggatacagttagagaattgaatggaggatcaggttcccctggtattcccctcagtctgatcaccgccgctgtgggtgccataataattctgtcactactgctcctccgccgttctaaacggggcaactcatctcatcctcctgggaattcagggcttccattcattggggagacattatcattcaccaaggcttttaaatcgaacacgctggaccaattttttgaggagagggtgaagaaattcgggcaagtctttaagctttccgtaatcgggcctcccacagtggcaatgtgcggccctgagggaaaccggtttgttttcgccaacgaggagaagcttgtccacttgtcgtggtctggtcgatatgcgaaaatcctgggtggagattccgtttccatgaagaggggagatgatcatcgcagagtacgtgccgcattcgcagggtttttgagccctgcatcactgcctgtttacataagtaaaatgagtgcacagatccaagatcatatcaacgaaaaatggaaagaaaaagttgtaattgctgtagttcctctggtaaaggagctcgtcttcaacgtttcctacaacttgtttttcagcataaatgatagcgaggaactgcatcgattgcataagattttcgaaactattgtggagggacatgtttccatgccgatagaccttcccggattcacctttcatagagcacttcagggaagggcgaagctcaagaaagttttctcttctttaatagaaaggagaagaagcgatctgagctccggattggcatctgctaatcaggatctcatctctgttttactcacctacaaagatgatagggggtatacaatgacccacgacgagctcctcgacaactttctttcccttcttgaatcctcctatgattccgtcaattcaccaatggcctgcatttttaagcttttgtatgacaatccagaatgctatgaaaaagtagttcaagagcaattggggatactttctggtaagaaggaaggacaagaaatctcgtggaaggatctgagatccatgaaatacacatggcaagtacttcaggaaacgctacgactgtatactcaagttgctggaatatttcgcaaagccatgactgacattcattatgatggtcacaccattcccaaagggtggcaacttctttgggcaacccaaactacacatctgaacgacaaatatttcagtgagccggaaaagttcatgccttccagattcgatgaagaaggaaacaatttgattccttactcattcgtaccatttggaggagggcggcggatgtgtccaggttgggaattcggaaagatggagatcttactctttgtccatcactttgttaaaacgttcagtggctttaccccaatcgatccggacgaaaaaattactgggaatccatttcctcatctccctgccaatggattttcaataaaacctactcccagatcctaa

SEQ ID NO: 62 - DNA, 1524 bp, unidentified
  source 1..1524: mol_type = other DNA; note = TOT10 reading frame nucleotide sequence; note (original language) = TOT10读码框核苷酸序列
atggttcatgtgttgcaggtagtgaaaatggatagagttagtgaaatatttaatggaagttcaggttctccagctggtattccccacagtgtgatcacagccggtgtgggtgccataataataattcttctgtcactagtgctcctccgccgttctagtaaacggggcgactcctctcatcctcctgggaattcaggccttccattcattggggagacattatcattcaccaaggcttttaaatcgaacacgctggccgaattttttgaggagagggtgaagaaattcgggaatgtatttaagatttcaataatcgggcctcccacagtggtaatgtgcggcaatgagggaaaccggtttattttcgccaacgaggagaagctgatgcacctgtcgtggtccggtcggtatgcgaaaatccttggtggggaatccgtttccatgaagaggggagatgatcatcgcagtgtacgtgccgcattcgcagggtttttgagcccttcggcgctgcctctttacgtagctaaaatgagtgcgcagatccaaaatcatatcaacgagaaatggaaaggaagagatgtaattgctgtagttcctttggtaaaagagctggtcttcaacgtttcctccaacttgtttttcagcatgaatgatagcgaggaattgcatctattgcatcaaattttcgaaactattgtagatggacatgtttccatgccgatagaccttcccggattcacctttcataaagcacttcagggaagggcgaagctcaagaaagtttactcttctttaatagaaaggagaagaagcgatctgagctccggattggcatctgctaatcaggatctcatctctgttttactcacctacaaagatgatagggggtatacaatgacccacgacgagctcctcgacaattttctttcccttattgaatcctcctatgattccatcaattcaccaatggcctgcatttttaagcttttgtatgccaatccagaatgctatgaaaaagtagttcaagagcaattggggatactttctggtaagaaggaaggagaagaaatctcatggaaggatctgagatccatgaaatacacatggcaagcaattcaggaaacgctacgaatttatactcaagttgcaggaatatttcgcaaagccatgactgacattcattatgatggtcacaccattcccaaagggtggcaacttctttgggcaacccaaactacacatctgaacgacaaatatttcagtgagcctgaaaaattcatgccttctagattcgatgaagaaggaaacaatgtgattccttactcattcgtaccatttggaggagggcggcggatgtgtccaggttgggaattcggaaagatggagatcttactctttgtccatcactttgttaaaacgttcagtggctttaccccaattgatccgaacgaaaaaattactgggaatccttttcctcatctccctgccaatggatttctaataaaacctattctcagatcctaa

SEQ ID NO: 63 - DNA, 1482 bp, unidentified
  source 1..1482: mol_type = other DNA; note = TOT11 reading frame nucleotide sequence; note (original language) = TOT11读码框核苷酸序列
atggatacagttagagaattgaatggaggatcaggttcccctggtattcccctcagtctgatcaccgccgctgtgggtgccataataattctgtcactactgctcctccgccgttctaaacggggcaactcatctcatcctcctgggaattcagggcttccattcattggggagacattatcattcaccaaggcttttaaatcgaacacgctggaccaatttttcgaggagagggtgaagaaattcgggcaagtctttaagctttccgtaatcgggcctcccacagtggcaatgtgcggccctgagggaaaccggtttgttttcgccaacgaggagaagcttgtccacttgtcgtggtctggtcgatatgcgaaaatcctgggtggagattccgtttccatgaagaggggagatgatcatcgcagtgtacgtgccgcattcgcagggtttttgagccctgcatcgctgcctgtttacataagtaaaatgagtgcacagatccaagatcatatcaacgaaaaatggaaaggaaaagatgtaattgctgtagttcctctggtaaaggagctcgtcttcaacgtttcctacaacttgtttttcagcttaaatgatagcgaggaactgcatcgattgcataagattttcgaaactattgtggagggacatgtttccatgccgatagaccttcccggattcacctttcatagagcacttcagggaagggcgaagctcaagaaagttttctcttctttaatagaaaggagaagaagcgatcttagctccggattggcatctgctaatcaggatctcatttctgttttactcacctacaaagatgatagggggtatacaatgacccacgacgagctcctcgacaactttctttcccttcttgaagcctcctatgattccgtcaattcaccaatggcctgcatttttaagcttttgtatgacaatccagaatgctatgaaaaagtagttcaagagcaattggggatactttctggtaagaaggaaggacaagaaatctcgtggaaggatctgagatccatgaaatacacatggcaagtacttcaggaaacgctacgactgtatactcaagttgctggaatatttcgcaaagccatgactgacattcattatgatggtcacaccattcccaaagggtggcaacttctttgggcaacccaaactacacatctgaacgacaaatatttcagtgagccggaaaagttcatgccttccagattcgatgaagaaggaaacaatttgattccttattcattcgtaccatttggaggagggcggcggatgtgtccaggttgggaattcggaaagatggagatcttactctttgtccatcactttgttaaaacgttcagtggctttaccccaatcgatccggacgaaaaaattactgggaatccatttcctcatctccctgccaatggattttcaataaaacctactcccagatcctaa

SEQ ID NO: 64 - DNA, 1497 bp, unidentified
  source 1..1497: mol_type = other DNA; note = TOT12 reading frame nucleotide sequence; note (original language) = TOT12读码框核苷酸序列
atggatagagttagagaaatatttaatggaagttcaggttctccagctggtattccccacagtgtgatcacagccggtgtgggtgccataataataattcttctgtcactactgctcctccgccgttctagtaaacggggcgactcctctcatcctcctgggaattcaggccttccattcattggggagacattatcattcaccaaggcttttaaatcgaacacgctggccgaattttttgaggagagggtgaagaaattcgggaatgtatttaagatttcaataatcgggcctcccacagtggtaatgtgcggcaatgagggaaaccggtttattttcgccaacgaggagaagctgatgcacctgtcgtggtccggtcgatatgcgaaaatccttggtggggaatccgtttccatgaagaggggagatgatcatcgcagtgtacgtgccgcattcgcagggtttttgagctctgcatcgctgcctgtttacataagtaaaatgagtgcacagatccaagatcatatcaacgaaaaatggaaaggaaaagatgtaattgctgtagttcctctggtaaaggagctcgtcttcaacgtttcctacaacttgtttttcagcataaatgatagcgaggaactgcatcgattgcataagattttcgaaactattgtggagggacatctttccatgccgatagaccttcccggattcacctttcatagagcacttcagggaagggcgaagctcaagaaagttttctcttctttaatagaaaggagaagaagcgatctgagctccggattggcatctgctaatcaggatctcatttctgttttactcacctacaaagatgatagggggtatacaatgacccacgacgagctcctcgacaactttctttcccttcttgaaggctcctatgattccatcaattcaccaatggcctgcatttttaagcttttgtatgacaatccagaatgctatgaaaaagtagttcaagagcaattggggatactttctggtaagaaggaaggacaagaaatctcgtggaaggatctgagatccatgaaatacacatggcaagtacttcaggaaacgctacgactgtatactcaagttgctggaatatttcgcaaagccatgactgacattcattatgatggtcacaccattcccaaagggtggcaacttctttgggcaaaccaaactacacatctgaacgacaaatatttcagtgagcctgaaaaattcatgccttccagattcgatgaagaaggaaacaatatgattccttactcattcgtaccatttggaggagggcggcggatgtgtccaggttgggaattcggaaagatggagatcttactctttgtccatcactttgttaaaacgttcagtggctttaccccaattgatccgaacgaaaaaattactgggaatccttttcctcatctccctgccaatggatttctaataaaacctattctcagatcctaa

SEQ ID NO: 65 - DNA, 1497 bp, unidentified
  source 1..1497: mol_type = other DNA; note = TOT13 reading frame nucleotide sequence; note (original language) = TOT13读码框核苷酸序列
atggatagagttagtgaaatatttaatggaagttcaggttctccagctggtattccccacagtgtgatcacagccggtgtgggtgccataataataattcttctgtcactagtgctcctccgccgttctagtaaacggggcgactcctctcatcctcctgggaattcaggccttccattcattggggagacattatcattcaccaaggcttttaaatcgaacacgctggccgaattttttgaggagagggtgaagaaattcgggaatgtatttaagatttcaataatcgggcctcccacagtggtaatgtgcggcaatgagggaaaccggtttattttcgccaacgaggagaagctgatgcacctgtcgtggtccggtcggtatgcgaaaatccttggtggggaatccgtttccatgaagaggggagatgatcatcgcagtgtacgtgccgcattcgcagggtttttgagcccttcggcgctgcctctttacgtagctaaaatgagtgcgcagatccaaaatcatatcaacgagaaatggaaaggaagagatgtaattgctgtagttcctttggtaaaagagctggtcttcaacgtttcctccaacttgtttttcagcatgaatgatagcgaggaattgcatctattgcatcaaattttcgaaactattgtagatggacatgtttccatgccgatagaccttcccggattcacctttcataaagcacttcagggaagggcgaagctcaagaaagtttactcttctttaatagaaaggagaagaagcgatctgagctccggattggcatctgctaatcaggatctcatctctgttttactcacctacaaagatgatagggggtatacaatgacccacgacgagctcctcgacaattttctttcccttattgaatcctcctatgattccatcaattcaccaatggcctgcatttttaagcttttgtatgccaatccagaatgctatgaaaaagtagttcaagagcaattggggatactttctggtaagaaggaaggagaagaaatctcatggaaggatctgagatccatgaaatacacatggcaagcaattcaggaaacgctacgaatttatactcaagttgcaggaatatttcgcaaagccatgactgacattcattatgatggtcacaccattcccaaagggtggcaacttctttgggcaacccaaactacacatctgaacgacaaatatttcagtgagcctgaaaaattcatgccttctagattcgatgaagaaggaaacaatgtgattccttactcattcgtaccatttggaggagggcggcggatgtgtccaggttgggaattcggaaagatggagatcttactctttgtccatcactttgttaaaacgttcagtggctttaccccaattgatccgaacgaaaaaattactgggaatccttttcctcatctccctgccaatggatttctaataaaacctattctcagatcctaa

SEQ ID NO: 66 - DNA, 1524 bp, unidentified
  source 1..1524: mol_type = other DNA; note = TOT14 reading frame nucleotide sequence; note (original language) = TOT14读码框核苷酸序列
atggttcatgtgttgcaggtagtgaaaatggatagagttagagaaatatttaatggaagttcaggttctccagctggtattccccacagtgtgatcacagccggtgtgggtgccataataataattcttctgtcactactgctcctccgccgttctagtaaacggggcgactcctctcatcctcctgggaattcaggccttccattcattggggagacattatcattcaccaaggcttttaaatcgaacacgctggccgaattttttgaggagagggtgaagaaattcgggaatgtatttaagatttcaataatcgggcctcccacagtggtaatgtgcggcaatgagggaaaccggtttattttcgccaacgaggagaagctgatgcacctgtcgtggtccggtcgatatgcgaaaatccttggtggggaatccgtttccatgaagaggggagatgatcatcgcagtgtacgtgccgcattcgcagggtttttgagccctgcatcgctgcctatttacataagtaaaatgagtgcacagatccaagatcatatcaacaaaaaatggaaaggaaaagatgtaattgctgtagttcctctggtaaaggagctcgtcttcaacgtttcctacaacttgtttttcagcataaatgatagcgaggaacttcatcgattgcataagattttcgaaactattgtggagggacatgtttccatgccgatagaccttcccggattcacctttcatagagcacttcagggaagggcgaagctcaagaaagtttactcttctttaatagaaaggagaagaagcgatctgagctccggattggcatctgctaatcaggatcttatctctgttttactcacctacaaagatgatagggggtatagaatgacccacgacgagctcctcgacaactttctttcccttcttgaatcctcctatgattccgtcaattcaccaatggcctgcattttaaagcttttgtatgccaatccagaatgctatgaaaaagtagttcaagagcaattggggatactttctggtaagaaggaaggagaagaaatctcatggaaggatctgagatccatgaaatacacatggcaagtacttcaggaaacgctacgactgtatactcaagttgctggaatatttcgcaaagccatgactgacattcattatgatggtcacaccattcccaaagggtggcaacttctttgggcaacccaaactacacatctgaacgacaaatatttcagtgagcctgaaaaattcatgccttccagattcgatgaagaaggaaacaatgtgattccttactcattcgtaccatttggaggagggcggcggatgtgtccaggttgggaattcggaaagatggagatcttactctttgtccatcactttgttaaaacgttcagtggctttaccccaattgatccgaacgaaaaaattactgggaatccttttcctcatctccctgccaatggatttctaataaaacctattctcagatcctaa

SEQ ID NO: 67 - DNA, 1524 bp, unidentified
  source 1..1524: mol_type = other DNA; note = TOT15 reading frame nucleotide sequence; note (original language) = TOT15读码框核苷酸序列
atggttcatgtgttgcaggtagtgaaaatggatagagttagagaaatatttaatggaagttcaggttctccagctggtattccccacagtgtgatcacagccggtgtgggtgccataataataattcttctgtcactactgctcctccgccgttctagtaaacggggcgactcctctcatcctcctgggaattcaggccttccattcattggggagacattatcattcaccaaggcttttaaatcgaacacgctggccgaattttttgaggagagggtgaagaaattcgggaatgtatttaagatttcaataatcgggcctcccacagtggtaatgtgcggcaatgagggaaaccggtttattttcgccaacgaggagaagctgatgcacctgtcgtggtccggtcgatatgcgaaaatccttggtggggaatccgtttccatgaagaggggagatgatcatcgcagtgtacgtgccgcattcgcagggtttttgagcccttcggcgctgcctctttacgtagctaaaatgagtgcgcagatccaaaatcatatcaacgagaaatggaaaggaagagatgtaattgccgtagttcctttggtaaaagagctggtcttcaacgtttcctccaacttgtttttcagcatgaatgatagcgaggaactgcatcgattgcatcaaattttcgaaactattgtagatggacatgtttccatgcccatagaccttcccggattcacctttcataaagcacttcagggaagggcgaagctcaagaaagtttactcttctttaatagaaaggagaagaagcgatctgagctccggattggcatctgctaatcaggatcttatctctgttttactcacctacaaagatgatagggggtatagaatgacccacgacgagctcctcgacaactttctttcccttcttgaatcctcctatgattccgtcaattcaccaatggcctgcattttaaagcttttgtatgccaatccagaatgctatgaaaaagtagttcaagagcaattggggatactttctggtaagaaggaaggagaagaaatctcatggaaggatctgagatccatgaaatacacatggcaagtacttcaggaaacgctacgactgtatactcaagttgctggaatatttcgcaaagccatgactgacattcattatgatggtcacaccattcccaaagggtggcaacttctttgggcaacccaaactacacatctgaacgacaaatatttcagtgagcctgaaaaattcatgccttccagattcgatgaagaaggaaacaatgtgattccttactcattcgtaccatttggaggagggcggcggatgtgtccaggttgggaattcggaaagatggagatcttactctttgtccatcactttgttaaaacgttcagtggctttaccccaattgatccgaacgaaaaaattactgggaatccttttcctcatctccctgccaatggatttctaataaaacctattctcagatcctaa

SEQ ID NO: 68 - DNA, 1497 bp, unidentified
  source 1..1497: mol_type = other DNA; note = TOT16 reading frame nucleotide sequence; note (original language) = TOT16读码框核苷酸序列
atggatagagttagagaaatatttaatggaagttcaggttctccagctggtattccccacagtgtgatcacagccggtgtgggtgccataataataattcttctgtcactactgctcctccgccgttctagtaaacggggcgactcctctcatcctcctgggaattcaggccttccattcattggggagacattatcattcaccaaggcttttaaatcgaacacgctggccgaattttttgaggagagggtgaagaaattcgggaatgtatttaagatttcaataatcgggcctcccacagtggtaatgtgcggcaatgagggaaaccggtttattttcgccaacgaggagaagctgatgcacctgtcgtggtccggtcgatatgcgaaaatccttggtggggaatccgtttccatgaagaggggagatgatcatcgcagtgtacgtgccgcattcgcagggtttttgagccctgcatcgctgcctatttacataagtaaaatgagtgcacagatccaagatcatatcaacaaaaaatggaaaggaaaagatgtaattgctgtagttcctctggtaaaggagctcgtcttcaacgtttcctacaacttgtttttcagcataaatgatagcgaggaacttcatcgattgcataagattttcgaaactattgtggagggacatgtttccatgccgatagaccttcccggattcacctttcatagagcacttcagggaagggcgaagctcaagaaagtttactcttctttaatagaaaggagaagaagcgatctgagctccggattggcatctgctaatcaggatcttatctctgttttactcacctacaaagatgatagggggtatagaatgacccacgacgagctcctcgacaactttctttcccttcttgaatcctcctatgattccgtcaattcaccaatggcctgcattttaaagcttttgtatgccaatccagaatgctatgaaaaagtagttcaagagcaattggggatactttctggtaagaaggaaggagaagaaatctcatggaaggatctgagatccatgaaatacacatggcaagtacttcaggaaacgctacgactgtatactcaagttgctggaatatttcgcaaagccatgactgacattcattatgatggtcacaccattcccaaagggtggcaacttctttgggcaacccaaactacacatctgaacgacaaatatttcagtgagcctgaaaaattcatgccttccagattcgatgaagaaggaaacaatgtgattccttactcattcgtaccatttggaggagggcggcggatgtgtccaggttgggaattcggaaagatggagatcttactctttgtccatcactttgttaaaacgttcagtggctttaccccaattgatccgaacgaaaaaattactgggaatccttttcctcatctccctgccaatggatttctaataaaacctattctcagatcctaa

SEQ ID NO: 69 - DNA, 1497 bp, unidentified
  source 1..1497: mol_type = other DNA; note = TOT17 reading frame nucleotide sequence; note (original language) = TOT17读码框核苷酸序列
atggatagagttagagaaatatttaatggaagttcaggttctccagctggtattccccacagtgtgatcacagccggtgtgggtgccataataataattcttctgtcactactgctcctccgccgttctagtaaacggggcgactcctctcatcctcctgggaattcaggccttccattcattggggagacattatcattcaccaaggcttttaaatcgaacacgctggccgaattttttgaggagagggtgaagaaattcgggaatgtatttaagatttcaataatcgggcctcccacagtggtaatgtgcggcaatgagggaaaccggtttattttcgccaacgaggagaagctgatgcacctgtcgtggtccggtcgatatgcgaaaatccttggtggggaatccgtttccatgaagaggggagatgatcatcgcagtgtacgtgccgcattcgcagggtttttgagcccttcggcgctgcctctttacgtagctaaaatgagtgcgcagatccaaaatcatatcaacgagaaatggaaaggaagagatgtaattgccgtagttcctttggtaaaagagctggtcttcaacgtttcctccaacttgtttttcagcatgaatgatagcgaggaactgcatcgattgcatcaaattttcgaaactattgtagatggacatgtttccatgcccatagaccttcccggattcacctttcataaagcacttcagggaagggcgaagctcaagaaagtttactcttctttaatagaaaggagaagaagcgatctgagctccggattggcatctgctaatcaggatcttatctctgttttactcacctacaaagatgatagggggtatagaatgacccacgacgagctcctcgacaactttctttcccttcttgaatcctcctatgattccgtcaattcaccaatggcctgcattttaaagcttttgtatgccaatccagaatgctatgaaaaagtagttcaagagcaattggggatactttctggtaagaaggaaggagaagaaatctcatggaaggatctgagatccatgaaatacacatggcaagtacttcaggaaacgctacgactgtatactcaagttgctggaatatttcgcaaagccatgactgacattcattatgatggtcacaccattcccaaagggtggcaacttctttgggcaacccaaactacacatctgaacgacaaatatttcagtgagcctgaaaaattcatgccttccagattcgatgaagaaggaaacaatgtgattccttactcattcgtaccatttggaggagggcggcggatgtgtccaggttgggaattcggaaagatggagatcttactctttgtccatcactttgttaaaacgttcagtggctttaccccaattgatccgaacgaaaaaattactgggaatccttttcctcatctccctgccaatggatttctaataaaacctattctcagatcctaa

SEQ ID NO: 70 - DNA, 1524 bp, unidentified
  source 1..1524: mol_type = other DNA; note = TOT18 reading frame nucleotide sequence; note (original language) = TOT18读码框核苷酸序列
atggttcatgtgttgcaggtagtgaaaatggatagagtcagtgaaatatttaatggaagttcaggttctccagctggtattccccacagtgtgatcacagccggtgtgggtgccataataataattcttctgtcactactgctcctccgccgttctagtaaacggggcgactcctctcatcctcctgggaattcaggccttccattcattggggagacattatcattcaccaaggcttttaaatcgaacacgctggccgaattttttgaggagagggtgaagaaattcgggaatgtatttaagatttcaataatcgggcctcccacagtggtaatgtgcggcaatgagggaaaccggtttattttcgccaacgaggagaagctgatgcacctgtcgtggtccggtcgatatgcgaaaatccttggtggggaatccgtttccatgaagaggggagatgatcatcgcagtgtacgtgccgcattcgcagggtttttgagcccttcggcgctgcctctttacgtagctaaaatgagtgcgcagatccaaaatcatatcaacgagaaatggaaaggaagagatgtaattgccgtagttcctttggtaaaagagctggtcttcaacgtttcctccaacttgtttttcagcatgaatgatagcgaggaactgcatcgattgcatcaaattttcgaaactattgtagatggacatgtttccatgcccatagaccttcccggattcacctttcataaagcacttcagggaagggcgaagctcaagaaagtttactcttctttaatagaaaggagaagaagcgatctgagctccggattggcatctgctaatcaggatctcatctctgttttactcacctacaaagatgatagggggtatacaatgacccatgacgagctcctcgacaattttctttcccttattgaatcctcctatgattccatcaattcaccaatggcctgcatttttaagcttttgtatgccaatccagaatgctatgaaaaagtagttcaagagcaattggggatactttctggtaagaaggaaggagaagaaatctcatggaaggatctgagatccatgaaatacacatggcaagcaattcaggaaacgctacgaatttatactcaagttgcaggaatatttcgcaaagccatgactgacattcattatgatggtcacaccattcccaaagggtggcaacttctttgggcaacccaaactacacatctgaacgacaaatatttcagtgagcctgaaaaattcatgccttccagattcgatgaagaaggaaacaatgtgattccttactcattcgtaccatttggaggagggcggcggatgtgtccaggttgggaattcggaaagatggagatcttactctttgtccatcactttgttaaaacgttcagtggctttaccccaattgatccgaacgaaaaaattactgggaatccttttcctcatctccctgccaatggatttctaataaaacctattctcagatcctaa

SEQ ID NO: 71 - DNA, 1494 bp, unidentified
  source 1..1494: mol_type = other DNA; note = TOT19 reading frame nucleotide sequence; note (original language) = TOT19读码框核苷酸序列
atggatgtcttttatccgttaaaaagtgcagtaacaaaatttaacgaatgtttccctgctattcttttcattgtcctcagtgctgttgctggcattgttctgcccctgctgctgttcctacgttctaaacgccgttcctctgttggactacccccagggaaattaggttaccctttcattggcgagtcgttactgttcctgaaggctcttcgatcaaacacagttgagcaatttttggacgagagagtgaagaaattcgggaatgtcttcaagacgtcattaattgggcatccgacagtagttctctgcgggcctgcgggaaaccggctaatcctggcgaacgaggagaagctggtgcagatgtcgtggcccaaatcctctatgaaactcatgggggaaaagtctatcaccgccaaaaggggcgaaggccatatgatcatccgctccgcactgcaaggctttttcagccctggtgctctgcagaaatacataggccaaatgagtaaaacaatagaaaatcatattaatgagaaatggaagggcaacgaccaagtgagtgtagttgctttggtaggagatctcgtcttcgatatatcggcctgtttgttcttcaatataaatgagaagcatgaacgggaacgactgtttgagcttttggagattatagctgtcggagttttggctgttccggtggatcttcccggatttgcttaccgtcgggcacttcaagcacggtcgaagcttaatgcaattctctccggtttgatagaaaagagaaaaatggatctgagctcaggattagcgagtagcaatcaggatcttctttctgtgtttctcaccttcaaagatgacagaggaaatccactgagcgatgaggaaatcctcgacaacttttccgggctgcttcatggatcctatgacaccactgtttcagcaatggcctgcgtttttaagcttttgtcttccaatcccgaatgctatgaaaaagtagttcaagagcaattggggatactttctggtaagaaggaaggacaagaaatctcgtggaaggatctgagatccatgaaatacacatggcaagtacttcaggaaacgctacgactgtatactcaagttgctggaatatttcgcaaagccatgactgacattcattatgatggtcacaccattcccaaagggtggcaacttctttgggcaacccaaactacacatctgaacgacaaatatttcagtgagccggaaaaattcatgccttccagattcgatgaagaaggaaacaatgtgattccttactcattcgtaccatttggaggagggcggcggatgtgtccaggttgggaattcggaaagatggagatcttactcttcgtccatcactttgttaaagcgttcagtggctttaccccaatcgatccggacgaaaaaattactgggaatccttttcctcatctccctgccaatggatttctaataaaacctattctcagatcctaa

SEQ ID NO: 72 - DNA, 1497 bp, unidentified
  source 1..1497: mol_type = other DNA; note = TOT20 reading frame nucleotide sequence; note (original language) = TOT20读码框核苷酸序列
atggatagagtcagtgaaatatttaatggaagttcaggttctccagctggtattccccacagtgtgatcacagccggtgtgggtgccataataataattcttctgtcactactgctcctccgccgttctagtaaacggggcgactcctctcatcctcctgggaattcaggccttccattcattggggagacattatcattcaccaaggcttttaaatcgaacacgctggccgaattttttgaggagagggtgaagaaattcgggaatgtatttaagatttcaataatcgggcctcccacagtggtaatgtgcggcaatgagggaaaccggtttattttcgccaacgaggagaagctgatgcacctgtcgtggtccggtcgatatgcgaaaatccttggtggggaatccgtttccatgaagaggggagatgatcatcgcagtgtacgtgccgcattcgcagggtttttgagcccttcggcgctgcctctttacgtagctaaaatgagtgcgcagatccaaaatcatatcaacgagaaatggaaaggaagagatgtaattgccgtagttcctttggtaaaagagctggtcttcaacgtttcctccaacttgtttttcagcatgaatgatagcgaggaactgcatcgattgcatcaaattttcgaaactattgtagatggacatgtttccatgcccatagaccttcccggattcacctttcataaagcacttcagggaagggcgaagctcaagaaagtttactcttctttaatagaaaggagaagaagcgatctgagctccggattggcatctgctaatcaggatctcatctctgttttactcacctacaaagatgatagggggtatacaatgacccatgacgagctcctcgacaattttctttcccttattgaatcctcctatgattccatcaattcaccaatggcctgcatttttaagcttttgtatgccaatccagaatgctatgaaaaagtagttcaagagcaattggggatactttctggtaagaaggaaggagaagaaatctcatggaaggatctgagatccatgaaatacacatggcaagcaattcaggaaacgctacgaatttatactcaagttgcaggaatatttcgcaaagccatgactgacattcattatgatggtcacaccattcccaaagggtggcaacttctttgggcaacccaaactacacatctgaacgacaaatatttcagtgagcctgaaaaattcatgccttccagattcgatgaagaaggaaacaatgtgattccttactcattcgtaccatttggaggagggcggcggatgtgtccaggttgggaattcggaaagatggagatcttactctttgtccatcactttgttaaaacgttcagtggctttaccccaattgatccgaacgaaaaaattactgggaatccttttcctcatctccctgccaatggatttctaataaaacctattctcagatcctaa

SEQ ID NO: 73 - DNA, 1524 bp, unidentified
  source 1..1524: mol_type = other DNA; note = TOT21 reading frame nucleotide sequence; note (original language) = TOT21读码框核苷酸序列
atggttcatgtgttgcaggtagtgaaaatggatagagttaatgaaatatttaatggaagttcaggttctccagctggtattccccacagtgtgatcacagccggtgtgggtgccataataataattcttctgtcactactgctcctccgccgttctagtaaacggggcgactccgctcatcctcctgggaattcaggccttccattcattggggagacattatcattcaccaaggcttttaaatcgaacacgctggccgaattttttgaggagagggtgaagaaattcgggaatgtatttaagatttcaataatcgggcctcccacagtggtaatgtgcggcaatgagggaaaccggtttattttcgccaacgaggagaagctgatgcacctgtcgtggtccggtcgatatgcgaaaatccttggtggggaatccgtttccatgaagaggggagatgatcatcgcagtgtacgtgccgcattcgcagggtttttgagctctgcatcgctgcctgtttacataagtaaaatgagtgcacagatccaagatcatatcaacgaaaaatggaaaggaaaagatgtaattgctgtagttcctctggtaaaggagctcgtcttcaacgtttcctacaacttgtttttcagcataaatgatagcgaggaactgcatcgattgcataagattttcgaaactattgtggagggacatgtttccatgccgatagaccttcccggattcacctttcatagagcacttcagggaagggagaagctcaagaaagttttctcttctttaatagaaaggagaagaagcgatcttagctccggattggcatctgctaatcaggatctcatttctgttttactcacctacaaagatgatagggggtatacaatgacccacgacgagctcctcgacaactttctttcccttcttgaatcctcctatgattccgtcaattcaccaatggcctgcatttttaagcttttgtatgacaatccagaatgctatgaaaaagtagttcaagagcaattggggatactttctggtaagaaggaaggacaagaaatctcgtggaaggatctgagatccatgaaatacacatggcaagtacttcaggaaacgctacgactgtatactcaagttgctggaatatttcgcaaagccatgactgacattcattatgatggtcacaccattcccaaagggtggcaacttctttgggcaacccaaactacacatctgaacgacaaatatttcagtgagccggaaaagttcatgccttccagattcggtgaagaaggaaacaatttgattccttactcattcgtaccatttggaggagggcggcggatgtgtccaggttgggaattcggaaagatggagatcttactctttgtccatcactttgttaaaacgttcagtggctttaccccaatcgatccggacgaaaaaattactgggaatccatttcctcatctccctgccaatggattttcaataaaacctactcccagatcctaa

SEQ ID NO: 74 - DNA, 1497 bp, unidentified
  source 1..1497: mol_type = other DNA; note = TOT22 reading frame nucleotide sequence; note (original language) = TOT22读码框核苷酸序列
atggatagagttaatgaaatatttaatggaagttcaggttctccagctggtattccccacagtgtgatcacagccggtgtgggtgccataataataattcttctgtcactactgctcctccgccgttctagtaaacggggcgactccgctcatcctcctgggaattcaggccttccattcattggggagacattatcattcaccaaggcttttaaatcgaacacgctggccgaattttttgaggagagggtgaagaaattcgggaatgtatttaagatttcaataatcgggcctcccacagtggtaatgtgcggcaatgagggaaaccggtttattttcgccaacgaggagaagctgatgcacctgtcgtggtccggtcgatatgcgaaaatccttggtggggaatccgtttccatgaagaggggagatgatcatcgcagtgtacgtgccgcattcgcagggtttttgagctctgcatcgctgcctgtttacataagtaaaatgagtgcacagatccaagatcatatcaacgaaaaatggaaaggaaaagatgtaattgctgtagttcctctggtaaaggagctcgtcttcaacgtttcctacaacttgtttttcagcataaatgatagcgaggaactgcatcgattgcataagattttcgaaactattgtggagggacatgtttccatgccgatagaccttcccggattcacctttcatagagcacttcagggaagggagaagctcaagaaagttttctcttctttaatagaaaggagaagaagcgatcttagctccggattggcatctgctaatcaggatctcatttctgttttactcacctacaaagatgatagggggtatacaatgacccacgacgagctcctcgacaactttctttcccttcttgaatcctcctatgattccgtcaattcaccaatggcctgcatttttaagcttttgtatgacaatccagaatgctatgaaaaagtagttcaagagcaattggggatactttctggtaagaaggaaggacaagaaatctcgtggaaggatctgagatccatgaaatacacatggcaagtacttcaggaaacgctacgactgtatactcaagttgctggaatatttcgcaaagccatgactgacattcattatgatggtcacaccattcccaaagggtggcaacttctttgggcaacccaaactacacatctgaacgacaaatatttcagtgagccggaaaagttcatgccttccagattcggtgaagaaggaaacaatttgattccttactcattcgtaccatttggaggagggcggcggatgtgtccaggttgggaattcggaaagatggagatcttactctttgtccatcactttgttaaaacgttcagtggctttaccccaatcgatccggacgaaaaaattactgggaatccatttcctcatctccctgccaatggattttcaataaaacctactcccagatcctaa

SEQ ID NO: 75 - DNA, 1524 bp, unidentified
  source 1..1524: mol_type = other DNA; note = TOT23 reading frame nucleotide sequence; note (original language) = TOT23读码框核苷酸序列
atggttcatgtgttgcaggtagtgaaaatggatagagttagtgaaatatttaatggaagttcaggttctccagctggtattccccacagtgtgatcacagccggtgtgggtgccataataataattcttctgtcactagtgctcctccgccgttctagtaaacggggcgactcctctcatcctcctgggaattcaggccttccattcattggggagacattatcattcaccaaggcttttaaatcgaacacgctggccgaattttttgaggagagggtgaagaaattcgggaatgtatttaagatttcaataatcgggcctcccacagtggtaatgtgcggcaatgagggaaaccggtttattttcgccaacgaggagaagctgatgcacctgtcgtggtccggtcgatatgcgaaaatccttggtggggaatccgtttccatgaagaggggagatgatcatcgcagtgtacgtgccgcattcgcagggtttttgagcccttcggcgctgcctctttacgtagctaaaatgagtgcgcagatccaaaatcatatcaacgagaaatggaaaggaagagatgtaattgctgtagttcctttggtaaaagagctggtcttcaacgtttcctccaacttgtttttcggcatgaatgatagcgaggaactgcatcgattgcatcaaattttcgaaactattgtagatggacatgtttccatgccgatagaccttcccggattcacctttcataaagcacttcagggaagggcgaagctcaagaaagtttactcttctttaatagaaaggagaagaagcgatctgagctccggattggcatctgctaatcaggatctcatctctgttttactcacctacaaagatgatagggggtatacaatgacccacgtcgagctcctcgacaattttctttcccttattgaatcctcctatgattccatcaattcaccaatggcctgcatttttaagcttttgtatgccaatccagaatgctatgaaaaagtagttcaagagcaattggggatactctctggtaagaagaaaggagaagaaatctcatggaaggatctgagatccatgaaatacacatggcaagcaattcaggaaacgctacgaatttatactcaagttgcaggaatatttcgcaaagccatgactgacattcattatgatggtcacaccattcccaaagggtggcaacttctttgggcaacccaaactacacatctgaacgacaaatatttcagtgagcctgaaaaattcatgccttccagattcgatgaagaaggaaacaatgtgattccttactcattcgtaccatttggaggagggcggcggatgtgtccaggttgggaattcggaaagatggagatcttactctttgtccatcactttgttaaaacgttcagtggctttaccccaattgatccgaacgaaaaaattactgggaatccttttcctcatctccctgccaatggatttctaataaaacctattctcagatcctaa

SEQ ID NO: 76 - DNA, 1533 bp, unidentified
  source 1..1533: mol_type = other DNA; note = TOT24 reading frame nucleotide sequence; note (original language) = TOT24读码框核苷酸序列
atggattccttgcatcgtgtaatcaagatctctgcaatatttaatggagacaccaaactacactggtcctcccctgctgttttttctgttgccttcactgctgttgccggcatacttcttctgttactgctcctccgttctaaacgccgccactcctctctgaatcagtacaatcttcctcgtggaaattcaggcctccctttcgttggggagacgatatcattcctgagggcctttcgaggaaacagaattcaacaattcttcgacgagagagcgaaaaaattcggaaatgtcttcaggatttcgataactgggcctcccacggcagtactgtgcggctcagagggaaaccgctttattctctccaacgaggagaagctggtgcgggttgacatgtccggagcattttccaaactggctggtcgggattccgtcatgatgagaacgggcgaggagcatcgcaccatacgagcagctatggcaggttttttggcccctacagcgctacccatttacgtgggtaaaatgagtgcacagatccaaaatcatatcgatgaaaaatggaaaggaaaagatgtggttactgtagtttctctcgtaaaagagctggtcttcggcgtttcagccagcatgttttacgatataaatgatggtgtcgaacagcatcgactgcacgagatttaccaaactatggttgcgggccatttttcttttccgctagattttcccggattttcttttcatagagcagttcagggaaggcagaagctcaagaaaattttctcttctttaatagaaaagaggagaagcgatctgcgctcgggattagcatctagcaatcaagatctactctccgttttgctcacctacaaaaatgaaaaagggaatggactcacgcagggtgagctcaccgacaactttattaccatgctcgaagcctcttatgacaaccccgtttcagccatttcctgtattctcaagttcttgtattcccatcccgaagtgtatgaaaaagtagttcaagagcaattgggcatactttcaaataaagaggagggagacgaaatctcatggaaggatgttaaagccatgaaatacacatggcaagctgtccaggaaacgttacgaatgatttctccagtgattggaatactgagaaaggccatgacagacattcattatgatggctacacaattccgaaaggatggcaactcctatggacaggctgcagtacacatctgaaagatgcatattttaatgaggcggacgaattcatgccttcaagattcgatgaggaaggaaagaatgtggttccttactcgtttgtgccatttggaggagggcgtcggatgtgtccaggatgggaattctctaaactggcgatactactgttcgtccatcactttgttaaaacattcagtagttacaccccacttgatcccgacgaaaaaattcttgggaatccattccctctcctccctgtcaatggactttccattaaacttactgccagatctgaaattaagaattaa

SEQ ID NO: 77 - DNA, 53 bp, synthetic construct
  source 1..53: mol_type = other DNA; note = P1 primer sequence
gtatattctgcccaaattcgcgaatggattccttaagttttctaaaaagcatg

SEQ ID NO: 78 - DNA, 57 bp, synthetic construct
  source 1..57: mol_type = other DNA; note = P2 primer sequence; note (original language) = P2引物序列
tgaaaccagagttaaaggcctcgagttaggttctgggaaatagtttaatgggaaatc

SEQ ID NO: 79 - DNA, 43 bp, synthetic construct
  source 1..43: mol_type = other DNA; note = P3 primer sequence; note (original language) = P3引物序列
gtatattctgcccaaattcgcgaatggttcatgtgttgcacgt

SEQ ID NO: 80 - DNA, 57 bp, synthetic construct
  source 1..57: mol_type = other DNA; note = P4 primer sequence; note (original language) = P4引物序列
accagagttaaaggcctcgagttaggatctgagaataggttttattagaaatccatt